European Patent Application EP 4 342 986 A1, published March 27, 2024. Title: Composition and method for treating LCA10 using RNA-guided Nuclease. Applicant: Genkore Korea Research Institute of Bioscience and Biotechnology. The sequence listing filed with the application follows.

SEQUENCE LISTING (492 sequences)

SEQ ID NO: 1 - DNA, 20 bp, Homo sapiens
taaataggcataattttcta

SEQ ID NO: 2 - DNA, 20 bp, Homo sapiens
ttgctttctgctgcttttgc

SEQ ID NO: 3 - DNA, 20 bp, Homo sapiens
gtagctttcaggattcctac

SEQ ID NO: 4 - DNA, 20 bp, Homo sapiens
ggagcttgttctgtcctcag

SEQ ID NO: 5 - DNA, 20 bp, Homo sapiens
gtttaacgttatcattttcc

SEQ ID NO: 6 - DNA, 20 bp, Homo sapiens
gctcatagagacacattcag

SEQ ID NO: 7 - DNA, 20 bp, Homo sapiens
tttctgatgaggaagatgaa

SEQ ID NO: 8 - DNA, 20 bp, Homo sapiens
gatcttagataagaataatc

SEQ ID NO: 9 - DNA, 20 bp, Homo sapiens
ttacttctaaataatattga

SEQ ID NO: 10 - DNA, 20 bp, Homo sapiens
tggaccatggatgcactctg

SEQ ID NO: 11 - DNA, 20 bp, Homo sapiens
gctacatccattccaaggaa

SEQ ID NO: 12 - DNA, 20 bp, Homo sapiens
ttttctcttagatgtctggt

SEQ ID NO: 13 - DNA, 20 bp, Homo sapiens
tgtagaattttaatgtagaa

SEQ ID NO: 14 - DNA, 20 bp, Homo sapiens
tcttacccctgtacccagaa

SEQ ID NO: 15 - DNA, 20 bp, Homo sapiens
cttgcatgatttagctgaat

SEQ ID NO: 16 - DNA, 20 bp, Homo sapiens
cagaagtcattcagccacta

SEQ ID NO: 17 - DNA, 20 bp, Homo sapiens
gtgtgtgtgttatgtgggaa

SEQ ID NO: 18 - DNA, 20 bp, Homo sapiens
ttattcattcagtttagtta

SEQ ID NO: 19 - DNA, 20 bp, Homo sapiens
gggatttggcagattttaat

SEQ ID NO: 20 - DNA, 20 bp, Homo sapiens
ctgccaaatccccccaaaca

SEQ ID NO: 21 - DNA, 20 bp, Homo sapiens
cacaaggttcaagaatcaca

SEQ ID NO: 22 - DNA, 20 bp, Homo sapiens
catcattttttattgtagaa

SEQ ID NO: 23 - DNA, 21 bp, Homo sapiens
gaatgtgtctctatgagccag

SEQ ID NO: 24 - DNA, 21 bp, Homo sapiens
taagatctaattctattagct

SEQ ID NO: 25 - DNA, 20 bp, Homo sapiens
tctcatgaacctttacctct

SEQ ID NO: 26 - DNA, 20 bp, Homo sapiens
tattagcttgaactctgtgc

SEQ ID NO: 27 - DNA, 20 bp, Homo sapiens
cattaaggaagacagatatg

SEQ ID NO: 28 - DNA, 20 bp, Homo sapiens
caggagtgactttgttccat

SEQ ID NO: 29 - DNA, 20 bp, Homo sapiens
gctaccggttacctgaaggg

SEQ ID NO: 30 - DNA, 20 bp, Homo sapiens
tgccacaagaatgatcattc

SEQ ID NO: 31 - DNA, 20 bp, Homo sapiens
tcccatgtgactccccgcct

SEQ ID NO: 32 - DNA, 20 bp, Homo sapiens
tattgttgctttttgagagg

SEQ ID NO: 33 - DNA, 20 bp, Homo sapiens
gtgaatttctattcctgttt

SEQ ID NO: 34 - DNA, 20 bp, Homo sapiens
gcatactttttttaatggaa

SEQ ID NO: 35 - DNA, 20 bp, Homo sapiens
ctcaacacacagaaacaaat

SEQ ID NO: 36 - DNA, 20 bp, Homo sapiens
gaatagataataaggaaata

SEQ ID NO: 37 - DNA, 20 bp, Homo sapiens
tttcttttttcttctactat

SEQ ID NO: 38 - DNA, 20 bp, Homo sapiens
cctgtgtttcaaggggatct

SEQ ID NO: 39 - DNA, 20 bp, Homo sapiens
cccttgaaacacaggaattg

SEQ ID NO: 40 - DNA, 20 bp, Homo sapiens
taagcaatggatttcagtga

SEQ ID NO: 41 - DNA, 20 bp, Homo sapiens
caatggatttcagtgataaa

SEQ ID NO: 42 - DNA, 20 bp, Homo sapiens
tattttccaggtactccact

SEQ ID NO: 43 - DNA, 20 bp, Homo sapiens
tacaaacagggtaatgagac

SEQ ID NO: 44 - DNA, 20 bp, Homo sapiens
tcctgtgtattcatagtata

SEQ ID NO: 45 - DNA, 20 bp, Homo sapiens
gataatcctattgtttgtta

SEQ ID NO: 46 - DNA, 20 bp, Homo sapiens
cactctctccctagtaactc

SEQ ID NO: 47 - DNA, 20 bp, Homo sapiens
gaaacttcactggtctcctt

SEQ ID NO: 48 - DNA, 20 bp, Homo sapiens
ctggcggattacctgagatc

SEQ ID NO: 49 - DNA, 20 bp, Homo sapiens
ctataattatgtactttact

SEQ ID NO: 50 - DNA, 20 bp, Homo sapiens
catgttggccgggctggtct

SEQ ID NO: 51 - RNA, 20 nt, Artificial Sequence
  Guide sequence for CRISPR/Cas12f1 system
uagaaaauuaugccuauuua

SEQ ID NO: 52 - RNA, 20 nt, Artificial Sequence
  Guide sequence for CRISPR/Cas12f1 system
gcaaaagcagcagaaagcaa

SEQ ID NO: 53 - RNA, 20 nt, Artificial Sequence
  Guide sequence for CRISPR/Cas12f1 system
guaggaauccugaaagcuac

SEQ ID NO: 54 - RNA, 20 nt, Artificial Sequence
  Guide sequence for CRISPR/Cas12f1 system
cugaggacagaacaagcucc

SEQ ID NO: 55 - RNA, 20 nt, Artificial Sequence
  Guide sequence for CRISPR/Cas12f1 system
ggaaaaugauaacguuaaac

SEQ ID NO: 56 - RNA, 20 nt, Artificial Sequence
  Guide sequence for CRISPR/Cas12f1 system
cugaaugugucucuaugagc

SEQ ID NO: 57 - RNA, 20 nt, Artificial Sequence
  Guide sequence for CRISPR/Cas12f1 system
uucaucuuccucaucagaaa

SEQ ID NO: 58 - RNA, 20 nt, Artificial Sequence
  Guide sequence for CRISPR/Cas12f1 system
gauuauucuuaucuaagauc

SEQ ID NO: 59 - RNA, 20 nt, Artificial Sequence
  Guide sequence for CRISPR/Cas12f1 system
ucaauauuauuuagaaguaa

SEQ ID NO: 60 - RNA, 20 nt, Artificial Sequence
  Guide sequence for CRISPR/Cas12f1 system
cagagugcauccauggucca

SEQ ID NO: 61 - RNA, 20 nt, Artificial Sequence
  Guide sequence for CRISPR/Cas12f1 system
uuccuuggaauggauguagc

SEQ ID NO: 62 - RNA, 20 nt, Artificial Sequence
  Guide sequence for CRISPR/Cas12f1 system
accagacaucuaagagaaaa

SEQ ID NO: 63 - RNA, 20 nt, Artificial Sequence
  Guide sequence for CRISPR/Cas12f1 system
uucuacauuaaaauucuaca

SEQ ID NO: 64 - RNA, 20 nt, Artificial Sequence
  Guide sequence for CRISPR/Cas12f1 system
uucuggguacagggguaaga

SEQ ID NO: 65 - RNA, 20 nt, Artificial Sequence
  Guide sequence for CRISPR/Cas12f1 system
auucagcuaaaucaugcaag

SEQ ID NO: 66 - RNA, 20 nt, Artificial Sequence
  Guide sequence for CRISPR/Cas12f1 system
uaguggcugaaugacuucug

SEQ ID NO: 67 - RNA, 20 nt, Artificial Sequence
  Guide sequence for CRISPR/Cas12f1 system
uucccacauaacacacacac

SEQ ID NO: 68 - RNA, 20 nt, Artificial Sequence
  Guide sequence for CRISPR/Cas12f1 system
uaacuaaacugaaugaauaa

SEQ ID NO: 69 - RNA, 20 nt, Artificial Sequence
  Guide sequence for CRISPR/Cas12f1 system
auuaaaaucugccaaauccc

SEQ ID NO: 70 - RNA, 20 nt, Artificial Sequence
  Guide sequence for CRISPR/Cas12f1 system
uguuuggggggauuuggcag

SEQ ID NO: 71 - RNA, 20 nt, Artificial Sequence
  Guide sequence for CRISPR/Cas12f1 system
ugugauucuugaaccuugug

SEQ ID NO: 72 - RNA, 20 nt, Artificial Sequence
  Guide sequence for CRISPR/Cas12f1 system
uucuacaauaaaaaaugaug

SEQ ID NO: 73 - RNA, 21 nt, Artificial Sequence
  Guide sequence for CRISPR/Cas12f1 system
cuggcucauagagacacauuc

SEQ ID NO: 74 - RNA, 21 nt, Artificial Sequence
  Guide sequence for CRISPR/Cas12f1 system
agcuaauagaauuagaucuua

SEQ ID NO: 75 - RNA, 20 nt, Artificial Sequence
  Guide sequence for CRISPR/Cas12f1 system
agagguaaagguucaugaga

SEQ ID NO: 76 - RNA, 20 nt, Artificial Sequence
  Guide sequence for CRISPR/Cas12f1 system
gcacagaguucaagcuaaua

SEQ ID NO: 77 - RNA, 20 nt, Artificial Sequence
  Guide sequence for CRISPR/Cas12f1 system
cauaucugucuuccuuaaug

SEQ ID NO: 78 - RNA, 20 nt, Artificial Sequence
  Guide sequence for CRISPR/Cas12f1 system
auggaacaaagucacuccug

SEQ ID NO: 79 - RNA, 20 nt, Artificial Sequence
  Guide sequence for CRISPR/Cas12f1 system
cccuucagguaaccgguagc

SEQ ID NO: 80 - RNA, 20 nt, Artificial Sequence
  Guide sequence for CRISPR/Cas12f1 system
gaaugaucauucuuguggca

SEQ ID NO: 81 - RNA, 20 nt, Artificial Sequence
  Guide sequence for CRISPR/Cas12f1 system
aggcggggagucacauggga

SEQ ID NO: 82 - RNA, 20 nt, Artificial Sequence
  Guide sequence for CRISPR/Cas12f1 system
ccucucaaaaagcaacaaua

SEQ ID NO: 83 - RNA, 20 nt, Artificial Sequence
  Guide sequence for CRISPR/Cas12f1 system
aaacaggaauagaaauucac

SEQ ID NO: 84 - RNA, 20 nt, Artificial Sequence
  Guide sequence for CRISPR/Cas12f1 system
uuccauuaaaaaaaguaugc

SEQ ID NO: 85 - RNA, 20 nt, Artificial Sequence
  Guide sequence for CRISPR/Cas12f1 system
auuuguuucuguguguugag

SEQ ID NO: 86 - RNA, 20 nt, Artificial Sequence
  Guide sequence for CRISPR/Cas12f1 system
uauuuccuuauuaucuauuc

SEQ ID NO: 87 - RNA, 20 nt, Artificial Sequence
  Guide sequence for CRISPR/Cas12f1 system
auaguagaagaaaaaagaaa

SEQ ID NO: 88 - RNA, 20 nt, Artificial Sequence
  Guide sequence for CRISPR/Cas12f1 system
agauccccuugaaacacagg

SEQ ID NO: 89 - RNA, 20 nt, Artificial Sequence
  Guide sequence for CRISPR/Cas12f1 system
caauuccuguguuucaaggg

SEQ ID NO: 90 - RNA, 20 nt, Artificial Sequence
  Guide sequence for CRISPR/Cas12f1 system
ucacugaaauccauugcuua

SEQ ID NO: 91 - RNA, 20 nt, Artificial Sequence
  Guide sequence for CRISPR/Cas12f1 system
uuuaucacugaaauccauug

SEQ ID NO: 92 - RNA, 20 nt, Artificial Sequence
  Guide sequence for CRISPR/Cas12f1 system
aguggaguaccuggaaaaua

SEQ ID NO: 93 - RNA, 20 nt, Artificial Sequence
  Guide sequence for CRISPR/Cas12f1 system
gucucauuacccuguuugua

SEQ ID NO: 94 - RNA, 20 nt, Artificial Sequence
  Guide sequence for CRISPR/Cas12f1 system
uauacuaugaauacacagga

SEQ ID NO: 95 - RNA, 20 nt, Artificial Sequence
  Guide sequence for CRISPR/Cas12f1 system
uaacaaacaauaggauuauc

SEQ ID NO: 96 - RNA, 20 nt, Artificial Sequence
  Guide sequence for CRISPR/Cas12f1 system
gaguuacuagggagagagug

SEQ ID NO: 97 - RNA, 20 nt, Artificial Sequence
  Guide sequence for CRISPR/Cas12f1 system
aaggagaccagugaaguuuc

SEQ ID NO: 98 - RNA, 20 nt, Artificial Sequence
  Guide sequence for CRISPR/Cas12f1 system
gaucucagguaauccgccag

SEQ ID NO: 99 - RNA, 20 nt, Artificial Sequence
  Guide sequence for CRISPR/Cas12f1 system
aguaaaguacauaauuauag

SEQ ID NO: 100 - RNA, 20 nt, Artificial Sequence
  Guide sequence for CRISPR/Cas12f1 system
agaccagcccggccaacaug

SEQ ID NO: 101 - RNA, 37 nt, Artificial Sequence
  Scaffold sequence of wildtype crRNA for CRISPR/Cas12f1 system
guugcagaacccgaauagacgaaugaaggaaugcaac

SEQ ID NO: 102 - RNA, 35 nt, Artificial Sequence
  Scaffold sequence of engineered crRNA for CRISPR/Cas12f1 system
ugcagaacccgaauagacgaaugaaggaaugcaac

SEQ ID NO: 103 - RNA, 33 nt, Artificial Sequence
  Scaffold sequence of engineered crRNA for CRISPR/Cas12f1 system
cagaacccgaauagacgaaugaaggaaugcaac

SEQ ID NO: 104 - RNA, 25 nt, Artificial Sequence
  Scaffold sequence of engineered crRNA for CRISPR/Cas12f1 system
gaauagacgaaugaaggaaugcaac

SEQ ID NO: 105 - RNA, 19 nt, Artificial Sequence
  Scaffold sequence of engineered crRNA for CRISPR/Cas12f1 system
acgaaugaaggaaugcaac

SEQ ID NO: 106 - RNA, 10 nt, Artificial Sequence
  Scaffold sequence of engineered crRNA for CRISPR/Cas12f1 system
ggaaugcaac

SEQ ID NO: 107 - RNA, 37 nt, Artificial Sequence
  Scaffold sequence of engineered crRNA for CRISPR/Cas12f1 system
guugcagaacccgaauagagcaaugaaggaaugcaac

SEQ ID NO: 108 - RNA, 25 nt, Artificial Sequence
  Scaffold sequence of engineered crRNA for CRISPR/Cas12f1 system
gaauagagcaaugaaggaaugcaac

SEQ ID NO: 109 - RNA, 19 nt, Artificial Sequence
  Scaffold sequence of engineered crRNA for CRISPR/Cas12f1 system
agcaaugaaggaaugcaac

SEQ ID NO: 110 - RNA, 161 nt, Artificial Sequence
  Scaffold sequence of wildtype tracrRNA for CRISPR/Cas12f1 system
cuucacugauaaaguggagaaccgcuucaccaaaagcugucccuuaggggauuagaacuugagugaaggugggcugcuugcaucagccuaaugucgagaagugcuuucuucggaaaguaacccucgaaacaaauucauuuuuccucuccaauucugcacaa

SEQ ID NO: 111 - RNA, 141 nt, Artificial Sequence
  Scaffold sequence of engineered tracrRNA for CRISPR/Cas12f1 system
accgcuucaccaaaagcugucccuuaggggauuagaacuugagugaaggugggcugcuugcaucagccuaaugucgagaagugcuuucuucggaaaguaacccucgaaacaaauucauuuuuccucuccaauucugcacaa

SEQ ID NO: 112 - RNA, 140 nt, Artificial Sequence
  Scaffold sequence of engineered tracrRNA for CRISPR/Cas12f1 system
cuucacugauaaaguggagaaccgcuucaccaaaagcugucccuuaggggauuagaacuugagugaaggugggcugcuugcaucagccuaaugucgagaagugcuuucuucggaaaguaacccucgaaacaaauucauuu

SEQ ID NO: 113 - RNA, 120 nt, Artificial Sequence
  Scaffold sequence of engineered tracrRNA for CRISPR/Cas12f1 system
accgcuucaccaaaagcugucccuuaggggauuagaacuugagugaaggugggcugcuugcaucagccuaaugucgagaagugcuuucuucggaaaguaacccucgaaacaaauucauuu

SEQ ID NO: 114 - RNA, 113 nt, Artificial Sequence
  Scaffold sequence of engineered tracrRNA for CRISPR/Cas12f1 system
accgcuucaccaaaagcugucccuuaggggauuagaacuugagugaaggugggcugcuugcaucagccuaaugucgagaagugcuuucuucggaaaguaacccucgaaacaaa

SEQ ID NO: 115 - RNA, 95 nt, Artificial Sequence
  Scaffold sequence of engineered tracrRNA for CRISPR/Cas12f1 system
accgcuucaccuuaggagugaaggugggcugcuugcaucagccuaaugucgagaagugcuuucuucggaaaguaacccucgaaacaaauucauuu

SEQ ID NO: 116 - RNA, 86 nt, Artificial Sequence
  Scaffold sequence of engineered tracrRNA for CRISPR/Cas12f1 system
accgcuucacuuagagugaaggugggcugcuugcaucagccuaaugucgagaagugcuuucuucggaaaguaacccucgaaacaaa

SEQ ID NO: 117 - RNA, 161 nt, Artificial Sequence
  Scaffold sequence of engineered tracrRNA for CRISPR/Cas12f1 system
cuucacugauaaaguggagaaccgcuucaccaaaagcugucccuuaggggauuagaacuugagugaaggugggcugcuugcaucagccuaaugucgagaagugcuuucuucggaaaguaacccucgaaacaaauucagugcuccucuccaauucugcacaa

SEQ ID NO: 118 - RNA, 141 nt, Artificial Sequence
  Scaffold sequence of engineered tracrRNA for CRISPR/Cas12f1 system
accgcuucaccaaaagcugucccuuaggggauuagaacuugagugaaggugggcugcuugcaucagccuaaugucgagaagugcuuucuucggaaaguaacccucgaaacaaauucagugcuccucuccaauucugcacaa

SEQ ID NO: 119 - RNA, 120 nt, Artificial Sequence
  Scaffold sequence of engineered tracrRNA for CRISPR/Cas12f1 system
accgcuucaccaauuaguugagugaaggugggcugcuugcaucagccuaaugucgagaagugcuuucuucggaaaguaacccucgaaacaaauucagugcuccucuccaauucugcacaa

SEQ ID NO: 120 - RNA, 107 nt, Artificial Sequence
  Scaffold sequence of engineered tracrRNA for CRISPR/Cas12f1 system
accgcuucaccaauuaguugagugaaggugggcugcuugcaucagccuaaugucgagaagugcuuucuucggaaaguaacccucgaaacaaauucagugcuccucuc

SEQ ID NO: 121 - RNA, 101 nt, Artificial Sequence
  Scaffold sequence of engineered tracrRNA for CRISPR/Cas12f1 system
accgcuucaccaauuaguugagugaaggugggcugcuugcaucagccuaaugucgagaagugcuuucuucggaaaguaacccucgaaacaaauucagugcu

SEQ ID NO: 122 - RNA, 202 nt, Artificial Sequence
  Scaffold region for CRISPR/Cas12f1 system
cuucacugauaaaguggagaaccgcuucaccaaaagcugucccuuaggggauuagaacuugagugaaggugggcugcuugcaucagccuaaugucgagaagugcuuucuucggaaaguaacccucgaaacaaauucauuuuuccucuccaauucugcacaagaaaguugcagaacccgaauagacgaaugaaggaaugcaac

SEQ ID NO: 123 - RNA, 202 nt, Artificial Sequence
  Scaffold region for CRISPR/Cas12f1 system
cuucacugauaaaguggagaaccgcuucaccaaaagcugucccuuaggggauuagaacuugagugaaggugggcugcuugcaucagccuaaugucgagaagugcuuucuucggaaaguaacccucgaaacaaauucagugcuccucuccaauucugcacaagaaaguugcagaacccgaauagacgaaugaaggaaugcaac

SEQ ID NO: 124 - RNA, 100 nt, Artificial Sequence
  Scaffold region for CRISPR/Cas12f1 system
accgcuucacuuagagugaaggugggcugcuugcaucagccuaaugucgagaagugcuuucuucggaaaguaacccucgaaacaaagaaaggaaugcaac

SEQ ID NO: 125 - RNA, 127 nt, Artificial Sequence
  Scaffold region for CRISPR/Cas12f1 system
accgcuucaccaaaagcugucccuuaggggauuagaacuugagugaaggugggcugcuugcaucagccuaaugucgagaagugcuuucuucggaaaguaacccucgaaacaaagaaaggaaugcaac

SEQ ID NO: 126 - RNA, 182 nt, Artificial Sequence
  Scaffold region for CRISPR/Cas12f1 system
accgcuucaccaaaagcugucccuuaggggauuagaacuugagugaaggugggcugcuugcaucagccuaaugucgagaagugcuuucuucggaaaguaacccucgaaacaaauucagugcuccucuccaauucugcacaagaaaguugcagaacccgaauagagcaaugaaggaaugcaac

SEQ ID NO: 127 - RNA, 10 nt, Artificial Sequence
  U-rich tail sequence
uuucuauuuu

SEQ ID NO: 128 - RNA, 10 nt, Artificial Sequence
  U-rich tail sequence
uuauguuuuu

SEQ ID NO: 129 - protein, 529 aa, Unknown
  Cas12f1 protein derived from Uncultured archaeon
MAKNTITKTLKLRIVRPYNSAEVEKIVADEKNNREKIALEKNKDKVKEACSKHLKVAAYCTTQVERNACLFCKARKLDDKFYQKLRGQFPDAVFWQEISEIFRQLQKQAAEIYNQSLIELYYEIFIKGKGIANASSVEHYLSDVCYTRAAELFKNAAIASGLRSKIKSNFRLKELKNMKSGLPTTKSDNFPIPLVKQKGGQYTGFEISNHNSDFIIKIPFGRWQVKKEIDKYRPWEKFDFEQVQKSPKPISLLLSTQRRKRNKGWSKDEGTEAEIKKVMNGDYQTSYIEVKRGSKIGEKSAWMLNLSIDVPKIDKGVDPSIIGGIDVGVKSPLVCAINNAFSRYSISDNDLFHFNKKMFARRRILLKKNRHKRAGHGAKNKLKPITILTEKSERFRKKLIERWACEIADFFIKNKVGTVQMENLESMKRKEDSYFNIRLRGFWPYAEMQNKIEFKLKQYGIEIRKVAPNNTSKTCSKCGHLNNYFNFEYRKKNKFPHFKCEKCNFKENADYNAALNISNPKLKSTKEEP

SEQ ID NO: 130 - protein, 7 aa, Artificial Sequence
  Nuclear Localization Sequence
PKKKRKV

SEQ ID NO: 131 - protein, 16 aa, Artificial Sequence
  Nuclear Localization Sequence
KRPAATKKAGQAKKKK

SEQ ID NO: 132 - protein, 9 aa, Artificial Sequence
  Nuclear Localization Sequence
PAAKRVKLD

SEQ ID NO: 133 - protein, 11 aa, Artificial Sequence
  Nuclear Localization Sequence
RQRRNELKRSP

SEQ ID NO: 134 - protein, 38 aa, Artificial Sequence
  Nuclear Localization Sequence
NQSSNFGPMKGGNFGGRSSGPYGGGGQYFAKPRNQGGY

SEQ ID NO: 135 - protein, 42 aa, Artificial Sequence
  Nuclear Localization Sequence
RMRIZFKNKGKDTAELRRRRVEVSVELRKAKKDEQILKRRNV

SEQ ID NO: 136 - protein, 8 aa, Artificial Sequence
  Nuclear Localization Sequence
VSRKRPRP

SEQ ID NO: 137 - protein, 8 aa, Artificial Sequence
  Nuclear Localization Sequence
PPKKARED

SEQ ID NO: 138 - protein, 8 aa, Artificial Sequence
  Nuclear Localization Sequence
PQPKKKPL

SEQ ID NO: 139 - protein, 12 aa, Artificial Sequence
  Nuclear Localization Sequence
SALIKKKKKMAP

SEQ ID NO: 140 - protein, 5 aa, Artificial Sequence
  Nuclear Localization Sequence
DRLRR

SEQ ID NO: 141 - protein, 7 aa, Artificial Sequence
  Nuclear Localization Sequence
PKQKKRK

SEQ ID NO: 142 - protein, 10 aa, Artificial Sequence
  Nuclear Localization Sequence
RKLKKKIKKL

SEQ ID NO: 143 - protein, 10 aa, Artificial Sequence
  Nuclear Localization Sequence
REKKKFLKRR

SEQ ID NO: 144 - protein, 20 aa, Artificial Sequence
  Nuclear Localization Sequence
KRKGDEVDGVDEVAKKKSKK

SEQ ID NO: 145 - protein, 17 aa, Artificial Sequence
  Nuclear Localization Sequence
RKCLQAGMNLEARKTKK

SEQ ID NO: 146 - DNA, 1587 bp, Artificial Sequence
  Human codon optimized nucleic acid encoding Cas12f1 protein
atggccaagaacacaattacaaagacactgaagctgaggatcgtgagaccatacaacagcgctgaggtcgagaagattgtggctgatgaaaagaacaacagggaaaagatcgccctcgagaagaacaaggataaggtgaaggaggcctgctctaagcacctgaaagtggccgcctactgcaccacacaggtggagaggaacgcctgtctgttttgtaaagctcggaagctggatgataagttttaccagaagctgcggggccagttccccgatgccgtcttttggcaggagattagcgagatcttcagacagctgcagaagcaggccgccgagatctacaaccagagcctgatcgagctctactacgagatcttcatcaagggcaagggcattgccaacgcctcctccgtggagcactacctgagcgacgtgtgctacacaagagccgccgagctctttaagaacgccgctatcgcttccgggctgaggagcaagattaagagtaacttccggctcaaggagctgaagaacatgaagagcggcctgcccactacaaagagcgacaacttcccaattccactggtgaagcagaaggggggccagtacacagggttcgagatttccaaccacaacagcgactttattattaagatcccctttggcaggtggcaggtcaagaaggagattgacaagtacaggccctgggagaagtttgatttcgagcaggtgcagaagagccccaagcctatttccctgctgctgtccacacagcggcggaagaggaacaaggggtggtctaaggatgaggggaccgaggccgagattaagaaagtgatgaacggcgactaccagacaagctacatcgaggtcaagcggggcagtaagattggcgagaagagcgcctggatgctgaacctgagcattgacgtgccaaagattgataagggcgtggatcccagcatcatcggagggatcgatgtgggggtcaagagccccctcgtgtgcgccatcaacaacgccttcagcaggtacagcatctccgataacgacctgttccactttaacaagaagatgttcgcccggcggaggattttgctcaagaagaaccggcacaagcgggccggacacggggccaagaacaagctcaagcccatcactatcctgaccgagaagagcgagaggttcaggaagaagctcatcgagagatgggcctgcgagatcgccgatttctttattaagaacaaggtcggaacagtgcagatggagaacctcgagagcatgaagaggaaggaggattcctacttcaacattcggctgagggggttctggccctacgctgagatgcagaacaagattgagtttaagctgaagcagtacgggattgagatccggaaggtggcccccaacaacaccagcaagacctgcagcaagtgcgggcacctcaacaactacttcaacttcgagtaccggaagaagaacaagttcccacacttcaagtgcgagaagtgcaactttaaggagaacgccgattacaacgccgccctgaacatcagcaaccctaagctgaagagcactaaggaggagccc

SEQ ID NO: 147 - DNA, 26 bp, Artificial Sequence
  Primer sequence
tgaactgactgctaagtacagggaca

SEQ ID NO: 148 - DNA, 20 bp, Artificial Sequence
  Primer sequence
aagcgttaagccgagatcgt

SEQ ID NO: 149 - DNA, 26 bp, Artificial Sequence
  Primer sequence
tgtggcagccattattcctgtctcta

SEQ ID NO: 150 - DNA, 26 bp, Artificial Sequence
  Primer sequence
tctgccttgactagctggttaggtaa

SEQ ID NO: 151 - DNA, 56 bp, Artificial Sequence
  Primer sequence
cactctttccctacacgacgctcttccgatctgaactgactgctaagtacagggac

SEQ ID NO: 152 - DNA, 61 bp, Artificial Sequence
  Primer sequence
gtgactggagttcagacgtgtgctcttccgatctgcaggcaaactttaattaaaatctgcc

SEQ ID NO: 153 - DNA, 54 bp, Artificial Sequence
  Primer sequence
cactctttccctacacgacgctcttccgatctggaacacctggaggtaagtttg

SEQ ID NO: 154 - DNA, 57 bp, Artificial Sequence
  Primer sequence
gtgactggagttcagacgtgtgctcttccgatctcattcagaagtcattcagccact

SEQ ID NO: 155 - DNA, 54 bp, Artificial Sequence
  Primer sequence
cactctttccctacacgacgctcttccgatctttgttcccacataacacacaca

SEQ ID NO: 156 - DNA, 60 bp, Artificial Sequence
  Primer sequence
gtgactggagttcagacgtgtgctcttccgatctttctgggtacaggggtaagagaaagg

SEQ ID NO: 157 - DNA, 53 bp, Artificial Sequence
  Primer sequence
cactctttccctacacgacgctcttccgatcttgtaatcaaaggagggaagca

SEQ ID NO: 158 - DNA, 58 bp, Artificial Sequence
  Primer sequence
gtgactggagttcagacgtgtgctcttccgatctgatgagaatttacagagtgcatcc

SEQ ID NO: 159 - DNA, 58 bp, Artificial Sequence
  Primer sequence
cactctttccctacacgacgctcttccgatctacccagaacaaactattctcccatgg

SEQ ID NO: 160 - DNA, 60 bp, Artificial Sequence
  Primer sequence
gtgactggagttcagacgtgtgctcttccgatctgggtctggtccatattcacagattgt

SEQ ID NO: 161 - DNA, 53 bp, Artificial Sequence
  Primer sequence
cactctttccctacacgacgctcttccgatcttggaccagaccctttgtagtt

SEQ ID NO: 162 - DNA, 56 bp, Artificial Sequence
  Primer sequence
gtgactggagttcagacgtgtgctcttccgatcttgtctctatgagccagcaaaag

SEQ ID NO: 163 - DNA, 60 bp, Artificial Sequence
  Primer sequence
cactctttccctacacgacgctcttccgatcttcatcttcctcatcagaaatagaggctt

SEQ ID NO: 164 - DNA, 60 bp, Artificial Sequence
  Primer sequence
gtgactggagttcagacgtgtgctcttccgatctgcaaaagcagcagaaagcaaactgat

SEQ ID NO: 165 - DNA, 58 bp, Artificial Sequence
  Primer sequence
cactctttccctacacgacgctcttccgatcttgctggctcatagagacacattcagt

SEQ ID NO: 166 - DNA, 58 bp, Artificial Sequence
  Primer sequence
gtgactggagttcagacgtgtgctcttccgatcttgctggagaggataggacagagga

SEQ ID NO: 167 - DNA, 53 bp, Artificial Sequence
  Primer sequence
cactctttccctacacgacgctcttccgatctttccattctccatgtcctctg

SEQ ID NO: 168 - DNA, 60 bp, Artificial Sequence
  Primer sequence
gtgactggagttcagacgtgtgctcttccgatctgggtgacagaatgaaactccatctca

SEQ ID NO: 169 - DNA, 52 bp, Artificial Sequence
  Primer sequence
cactctttccctacacgacgctcttccgatctgtggcagccattattcctgt

SEQ ID NO: 170 - DNA, 57 bp, Artificial Sequence
  Primer sequence
gtgactggagttcagacgtgtgctcttccgatctgaacactgtggtcagaaaactca

SEQ ID NO: 171 - DNA, 58 bp, Artificial Sequence
  Primer sequence
cactctttccctacacgacgctcttccgatctatgtatgttcttttgtacgtgctctt

SEQ ID NO: 172 - DNA, 64 bp, Artificial Sequence
  Primer sequence
gtgactggagttcagacgtgtgctcttccgatctaagacagatatgtaaacacatataatttga

SEQ ID NO: 173 - DNA, 58 bp, Artificial Sequence
  Primer sequence
cactctttccctacacgacgctcttccgatctgtcactcctgtctacactagttctgc

SEQ ID NO: 174 - DNA, 60 bp, Artificial Sequence
  Primer sequence
gtgactggagttcagacgtgtgctcttccgatctaccatatttgacaccacatgcactgt

SEQ ID NO: 175 - DNA, 59 bp, Artificial Sequence
  Primer sequence
cactctttccctacacgacgctcttccgatctttccttaatggaatataagtcttttga

SEQ ID NO: 176 - DNA, 62 bp, Artificial Sequence
  Primer sequence
gtgactggagttcagacgtgtgctcttccgatctccttattatctattccattcttcacaca

SEQ ID NO: 177 - DNA, 55 bp, Artificial Sequence
  Primer sequence
cactctttccctacacgacgctcttccgatctggttcatgagactagaggtcacg

SEQ ID NO: 178 - DNA, 54 bp, Artificial Sequence
  Primer sequence
gtgactggagttcagacgtgtgctcttccgatctctgggcaacacagtgagact

SEQ ID NO: 179 - DNA, 52 bp, Artificial Sequence
  Primer sequence
cactctttccctacacgacgctcttccgatctggttcaagcgattcttctgc

SEQ ID NO: 180 - DNA, 55 bp, Artificial Sequence
  Primer sequence
gtgactggagttcagacgtgtgctcttccgatctcctgaaacttcactggtctcc

SEQ ID NO: 181 - DNA, 52 bp, Artificial Sequence
  Primer sequence
cactctttccctacacgacgctcttccgatctagcctcaacttcccaaagtg

SEQ ID NO: 182 - DNA, 54 bp, Artificial Sequence
  Primer sequence
gtgactggagttcagacgtgtgctcttccgatcttctttttctcccacctaccc

SEQ ID NO: 183 - DNA, 60 bp, Artificial Sequence
  Primer sequence
cactctttccctacacgacgctcttccgatcttttagagttactagggagagagtgatga

SEQ ID NO: 184 - DNA, 54 bp, Artificial Sequence
  Primer sequence
gtgactggagttcagacgtgtgctcttccgatctacacaggagggaaaacagga

SEQ ID NO: 185 - DNA, 54 bp, Artificial Sequence
  Primer sequence
cactctttccctacacgacgctcttccgatcttcctgtgaaaaaggatgaaagg

SEQ ID NO: 186 - DNA, 61 bp, Artificial Sequence
  Primer sequence
gtgactggagttcagacgtgtgctcttccgatcttgaagaataatacaaacagggtaatga

SEQ ID NO: 187 - DNA, 52 bp, Artificial Sequence
  Primer sequence
cactctttccctacacgacgctcttccgatctctcctgttttccctcctgtg

SEQ ID NO: 188 - DNA, 55 bp, Artificial Sequence
  Primer sequence
gtgactggagttcagacgtgtgctcttccgatcttttgagtggagtacctggaaa

SEQ ID NO: 189 - DNA, 57 bp, Artificial Sequence
  Primer sequence
cactctttccctacacgacgctcttccgatcttgtcctctttttagtctcattaccc

SEQ ID NO: 190 - DNA, 55 bp, Artificial Sequence
  Primer sequence
gtgactggagttcagacgtgtgctcttccgatctggaaaaaggctggcgatataa

SEQ ID NO: 191 - DNA, 52 bp, Artificial Sequence
  Primer sequence
cactctttccctacacgacgctcttccgatctatatcgccagcctttttcct

SEQ ID NO: 192 - DNA, 56 bp, Artificial Sequence
  Primer sequence
gtgactggagttcagacgtgtgctcttccgatctgccttgactagctggttaggta

SEQ ID NO: 193 - DNA, 22 bp, Artificial Sequence
  Primer sequence
cttggctcactgcaagctccac

SEQ ID NO: 194 - DNA, 30 bp, Artificial Sequence
  Primer sequence
acagggtaggattcatgtttagaatgatca

SEQ ID NO: 195 - DNA, 20 bp, Homo sapiens
tagaaaattatgcctattta

SEQ ID NO: 196 - DNA, 20 bp, Homo sapiens
gcaaaagcagcagaaagcaa

SEQ ID NO: 197 - DNA, 20 bp, Homo sapiens
gtaggaatcctgaaagctac

SEQ ID NO: 198 - DNA, 20 bp, Homo sapiens
ctgaggacagaacaagctcc

SEQ ID NO: 199 - DNA, 20 bp, Homo sapiens
ggaaaatgataacgttaaac

SEQ ID NO: 200 - DNA, 20 bp, Homo sapiens
ctgaatgtgtctctatgagc

SEQ ID NO: 201 - DNA, 20 bp, Homo sapiens
ttcatcttcctcatcagaaa

SEQ ID NO: 202 - DNA, 20 bp, Homo sapiens
gattattcttatctaagatc

SEQ ID NO: 203 - DNA, 20 bp, Homo sapiens
tcaatattatttagaagtaa

SEQ ID NO: 204 - DNA, 20 bp, Homo sapiens
cagagtgcatccatggtcca

SEQ ID NO: 205 - DNA, 20 bp, Homo sapiens
ttccttggaatggatgtagc

SEQ ID NO: 206 - DNA, 20 bp, Homo sapiens
accagacatctaagagaaaa

SEQ ID NO: 207 - DNA, 20 bp, Homo sapiens
ttctacattaaaattctaca

SEQ ID NO: 208 - DNA, 20 bp, Homo sapiens
ttctgggtacaggggtaaga

SEQ ID NO: 209 - DNA, 20 bp, Homo sapiens
attcagctaaatcatgcaag

SEQ ID NO: 210 - DNA, 20 bp, Homo sapiens
tagtggctgaatgacttctg

SEQ ID NO: 211 - DNA, 20 bp, Homo sapiens
ttcccacataacacacacac

SEQ ID NO: 212 - DNA, 20 bp, Homo sapiens
taactaaactgaatgaataa

SEQ ID NO: 213 - DNA, 20 bp, Homo sapiens
attaaaatctgccaaatccc

SEQ ID NO: 214 - DNA, 20 bp, Homo sapiens
tgtttggggggatttggcag

SEQ ID NO: 215 - DNA, 20 bp, Homo sapiens
tgtgattcttgaaccttgtg

SEQ ID NO: 216 - DNA, 20 bp, Homo sapiens
ttctacaataaaaaatgatg

SEQ ID NO: 217 - DNA, 21 bp, Homo sapiens
ctggctcatagagacacattc

SEQ ID NO: 218 - DNA, 21 bp, Homo sapiens
agctaatagaattagatctta

SEQ ID NO: 219 - DNA, 20 bp, Homo sapiens
agaggtaaaggttcatgaga

SEQ ID NO: 220 - DNA, 20 bp, Homo sapiens
gcacagagttcaagctaata

SEQ ID NO: 221 - DNA, 20 bp, Homo sapiens
catatctgtcttccttaatg

SEQ ID NO: 222 - DNA, 20 bp, Homo sapiens
atggaacaaagtcactcctg

SEQ ID NO: 223 - DNA, 20 bp, Homo sapiens
cccttcaggtaaccggtagc

SEQ ID NO: 224 - DNA, 20 bp, Homo sapiens
gaatgatcattcttgtggca

SEQ ID NO: 225 - DNA, 20 bp, Homo sapiens
aggcggggagtcacatggga

SEQ ID NO: 226 - DNA, 20 bp, Homo sapiens
cctctcaaaaagcaacaata

SEQ ID NO: 227 - DNA, 20 bp, Homo sapiens
aaacaggaatagaaattcac

SEQ ID NO: 228 - DNA, 20 bp, Homo sapiens
ttccattaaaaaaagtatgc

SEQ ID NO: 229 - DNA, 20 bp, Homo sapiens
atttgtttctgtgtgttgag

SEQ ID NO: 230 - DNA, 20 bp, Homo sapiens
tatttccttattatctattc

SEQ ID NO: 231 - DNA, 20 bp, Homo sapiens
atagtagaagaaaaaagaaa

SEQ ID NO: 232 - DNA, 20 bp, Homo sapiens
agatccccttgaaacacagg

SEQ ID NO: 233 - DNA, 20 bp, Homo sapiens
caattcctgtgtttcaaggg

SEQ ID NO: 234 - DNA, 20 bp, Homo sapiens
tcactgaaatccattgctta

SEQ ID NO: 235 - DNA, 20 bp, Homo sapiens
tttatcactgaaatccattg

SEQ ID NO: 236 - DNA, 20 bp, Homo sapiens
agtggagtacctggaaaata

SEQ ID NO: 237 - DNA, 20 bp, Homo sapiens
gtctcattaccctgtttgta

SEQ ID NO: 238 - DNA, 20 bp, Homo sapiens
tatactatgaatacacagga

SEQ ID NO: 239 - DNA, 20 bp, Homo sapiens
taacaaacaataggattatc

SEQ ID NO: 240 - DNA, 20 bp, Homo sapiens
gagttactagggagagagtg

SEQ ID NO: 241 - DNA, 20 bp, Homo sapiens
aaggagaccagtgaagtttc

SEQ ID NO: 242 - DNA, 20 bp, Homo sapiens
gatctcaggtaatccgccag

SEQ ID NO: 243 - DNA, 20 bp, Homo sapiens
agtaaagtacataattatag

SEQ ID NO: 244 - DNA, 20 bp, Homo sapiens
agaccagcccggccaacatg

SEQ ID NO: 245 - RNA, 19 nt, Artificial Sequence
  Guide sequence for CRISPR/Cas12f1 system
cagagugcauccauggucc

SEQ ID NO: 246 - RNA, 21 nt, Artificial Sequence
  Guide sequence for CRISPR/Cas12f1 system
cagagugcauccaugguccag

SEQ ID NO: 247 - RNA, 22 nt, Artificial Sequence
  Guide sequence for CRISPR/Cas12f1 system
cagagugcauccaugguccagg

SEQ ID NO: 248 - RNA, 23 nt, Artificial Sequence
  Guide sequence for CRISPR/Cas12f1 system
cagagugcauccaugguccagga

SEQ ID NO: 249 - RNA, 24 nt, Artificial Sequence
  Guide sequence for CRISPR/Cas12f1 system
cagagugcauccaugguccaggaa

SEQ ID NO: 250 - RNA, 25 nt, Artificial Sequence
  Guide sequence for CRISPR/Cas12f1 system
cagagugcauccaugguccaggaag

SEQ ID NO: 251 - RNA, 19 nt, Artificial Sequence
  Guide sequence for CRISPR/Cas12f1 system
uucuggguacagggguaag

SEQ ID NO: 252 - RNA, 21 nt, Artificial Sequence
  Guide sequence for CRISPR/Cas12f1 system
uucuggguacagggguaagag

SEQ ID NO: 253 - RNA, 22 nt, Artificial Sequence
  Guide sequence for CRISPR/Cas12f1 system
uucuggguacagggguaagaga

SEQ ID NO: 254 - RNA, 23 nt, Artificial Sequence
  Guide sequence for CRISPR/Cas12f1 system
uucuggguacagggguaagagaa

SEQ ID NO: 255 - RNA, 24 nt, Artificial Sequence
  Guide sequence for CRISPR/Cas12f1 system
uucuggguacagggguaagagaaa

SEQ ID NO: 256 - RNA, 25 nt, Artificial Sequence
  Guide sequence for CRISPR/Cas12f1 system
uucuggguacagggguaagagaaag

SEQ ID NO: 257 - RNA, 19 nt, Artificial Sequence
  Guide sequence for CRISPR/Cas12f1 system
cccuucagguaaccgguag

SEQ ID NO: 258 - RNA, 25 nt, Artificial Sequence
  Guide sequence for CRISPR/Cas12f1 system
cccuucagguaaccgguagcuuuug

SEQ ID NO: 259 - RNA, 19 nt, Artificial Sequence
  Guide sequence for CRISPR/Cas12f1 system
aggcggggagucacauggg

SEQ ID NO: 260 - RNA, 21 nt, Artificial Sequence
  Guide sequence for CRISPR/Cas12f1 system
aggcggggagucacaugggag

SEQ ID NO: 261 - RNA, 23 nt, Artificial Sequence
  Guide sequence for CRISPR/Cas12f1 system
aggcggggagucacaugggaguc

SEQ ID NO: 262 - RNA, 24 nt, Artificial Sequence
  Guide sequence for CRISPR/Cas12f1 system
aggcggggagucacaugggaguca

SEQ ID NO: 263 - RNA, 25 nt, Artificial Sequence
  Guide sequence for CRISPR/Cas12f1 system
aggcggggagucacaugggagucac

SEQ ID NO: 264 - RNA, 21 nt, Artificial Sequence
  Guide sequence for CRISPR/Cas12f1 system
aguggaguaccuggaaaauaa

SEQ ID NO: 265 - RNA, 22 nt, Artificial Sequence
  Guide sequence for CRISPR/Cas12f1 system
aguggaguaccuggaaaauaag

SEQ ID NO: 266 - RNA, 23 nt, Artificial Sequence
  Guide sequence for CRISPR/Cas12f1 system
aguggaguaccuggaaaauaagc

SEQ ID NO: 267 - RNA, 24 nt, Artificial Sequence
  Guide sequence for CRISPR/Cas12f1 system
aguggaguaccuggaaaauaagcc

SEQ ID NO: 268 - RNA, 25 nt, Artificial Sequence
  Guide sequence for CRISPR/Cas12f1 system
aguggaguaccuggaaaauaagcca

SEQ ID NO: 269 - RNA, 21 nt, Artificial Sequence
  Guide sequence for CRISPR/Cas12f1 system
gaguuacuagggagagaguga

SEQ ID NO: 270 - RNA, 23 nt, Artificial Sequence
  Guide sequence for CRISPR/Cas12f1 system
gaguuacuagggagagagugaug

SEQ ID NO: 271 - RNA, 24 nt, Artificial Sequence
  Guide sequence for CRISPR/Cas12f1 system
gaguuacuagggagagagugauga

SEQ ID NO: 272 - RNA, 25 nt, Artificial Sequence
  Guide sequence for CRISPR/Cas12f1 system
gaguuacuagggagagagugaugaa

SEQ ID NO: 273 - DNA, 20 bp, Homo sapiens
atccctattggcagtgtctt

SEQ ID NO: 274 - DNA, 100 bp, Artificial Sequence
  Donor sequence for introducing a mutation using CRISPR/Cas9 system
gagccaccgcacctggccccagttgtaattgtgagtatctcatagatatccctattggcagtgtcttagttttattttttattatctttattgtggcagc

SEQ ID NO: 275 - DNA, 26 bp, Artificial Sequence
  Primer sequence
ccattttcaagattgcagctctccaa

SEQ ID NO: 276 - DNA, 26 bp, Artificial Sequence
  Primer sequence
tccaggtgttccaagttacttgttct

SEQ ID NO: 277 - DNA, 26 bp, Artificial Sequence
  Primer sequence
tgactgctaagtacagggacatcttg

SEQ ID NO: 278 - DNA, 26 bp, Artificial Sequence
  Primer sequence
atctgtaatcccagcactttaggagg

SEQ ID NO: 279 - DNA, 26 bp, Artificial Sequence
  Primer sequence
aggaaatggccattttcaagattgca

SEQ ID NO: 280 - DNA, 25 bp, Artificial Sequence
  Primer sequence
agactccacttgttcttttaaggag

SEQ ID NO: 281 - DNA, 26 bp, Artificial Sequence
  Primer sequence
tagagatggggtttcaccttgttagc

SEQ ID NO: 282 - DNA, 25 bp, Artificial Sequence
  Primer sequence
agactccacttgttcttttaaggag

SEQ ID NO: 283 - DNA, 32 bp, Homo sapiens
cctggccccagttgtaattgtgaatatctcat

SEQ ID NO: 284 - DNA, 32 bp, Artificial Sequence
  Mutation sequence
cctggccccagttgtaattgtgagtatctcat

SEQ ID NO: 285 - DNA, 32 bp, Artificial Sequence
  Mutation sequence
cctggccccaattgtaattgtgaatatctcat

SEQ ID NO: 286 - DNA, 69 bp, Homo sapiens
ctcctaaagtgctgggattacagatgtgagccaccgcacctggccccagttgtaattgtgaatatctca

SEQ ID NO: 287 - DNA, 69 bp, Artificial Sequence
  Mutation sequence
ctcctaaagtgctgggattacagatgtgagccaccgcacctggccccagttgtaattgtgagtatctca

SEQ ID NO: 288 - protein, 557 aa, Artificial Sequence
  TnpB
MGEKSSRRRRNGKSGAWTAAITSCVGGKMAKNTITKTLKLRIVRPYNSAEVEKIVADEKNNREKIALEKNKDKVKEACSKHLKVAAYCTTQVERNACLFCKARKLDDKFYQKLRGQFPDAVFWQEISEIFRQLQKQAAEIYNQSLIELYYEIFIKGKGIANASSVEHYLSDVCYTRAAELFKNAAIASGLRSKIKSNFRLKELKNMKSGLPTTKSDNFPIPLVKQKGGQYTGFEISNHNSDFIIKIPFGRWQVKKEIDKYRPWEKFDFEQVQKSPKPISLLLSTQRRKRNKGWSKDEGTEAEIKKVMNGDYQTSYIEVKRGSKIGEKSAWMLNLSIDVPKIDKGVDPSIIGGIDVGVKSPLVCAINNAFSRYSISDNDLFHFNKKMFARRRILLKKNRHKRAGHGAKNKLKPITILTEKSERFRKKLIERWACEIADFFIKNKVGTVQMENLESMKRKEDSYFNIRLRGFWPYAEMQNKIEFKLKQYGIEIRKVAPNNTSKTCSKCGHLNNYFNFEYRKKNKFPHFKCEKCNFKENADYNAALNISNPKLKSTKEEP

SEQ ID NO: 289 - protein, 555 aa, Artificial Sequence
  Cas12f1 + CasX 26aa
MEKRINKIRKKLSADNATKPVSRSGPMAKNTITKTLKLRIVRPYNSAEVEKIVADEKNNREKIALEKNKDKVKEACSKHLKVAAYCTTQVERNACLFCKARKLDDKFYQKLRGQFPDAVFWQEISEIFRQLQKQAAEIYNQSLIELYYEIFIKGKGIANASSVEHYLSDVCYTRAAELFKNAAIASGLRSKIKSNFRLKELKNMKSGLPTTKSDNFPIPLVKQKGGQYTGFEISNHNSDFIIKIPFGRWQVKKEIDKYRPWEKFDFEQVQKSPKPISLLLSTQRRKRNKGWSKDEGTEAEIKKVMNGDYQTSYIEVKRGSKIGEKSAWMLNLSIDVPKIDKGVDPSIIGGIDVGVKSPLVCAINNAFSRYSISDNDLFHFNKKMFARRRILLKKNRHKRAGHGAKNKLKPITILTEKSERFRKKLIERWACEIADFFIKNKVGTVQMENLESMKRKEDSYFNIRLRGFWPYAEMQNKIEFKLKQYGIEIRKVAPNNTSKTCSKCGHLNNYFNFEYRKKNKFPHFKCEKCNFKENADYNAALNISNPKLKSTKEEP

SEQ ID NO: 290 - protein, 557 aa, Artificial Sequence
  Cas12f1 + random 28aa
MAGGPGAGSAAPVSSTSSLPLAALNMRVMAKNTITKTLKLRIVRPYNSAEVEKIVADEKNNREKIALEKNKDKVKEACSKHLKVAAYCTTQVERNACLFCKARKLDDKFYQKLRGQFPDAVFWQEISEIFRQLQKQAAEIYNQSLIELYYEIFIKGKGIANASSVEHYLSDVCYTRAAELFKNAAIASGLRSKIKSNFRLKELKNMKSGLPTTKSDNFPIPLVKQKGGQYTGFEISNHNSDFIIKIPFGRWQVKKEIDKYRPWEKFDFEQVQKSPKPISLLLSTQRRKRNKGWSKDEGTEAEIKKVMNGDYQTSYIEVKRGSKIGEKSAWMLNLSIDVPKIDKGVDPSIIGGIDVGVKSPLVCAINNAFSRYSISDNDLFHFNKKMFARRRILLKKNRHKRAGHGAKNKLKPITILTEKSERFRKKLIERWACEIADFFIKNKVGTVQMENLESMKRKEDSYFNIRLRGFWPYAEMQNKIEFKLKQYGIEIRKVAPNNTSKTCSKCGHLNNYFNFEYRKKNKFPHFKCEKCNFKENADYNAALNISNPKLKSTKEEP

SEQ ID NO: 291 - protein, 555 aa, Artificial Sequence
  Cas12f1 + random 26aa
MAGGPGAGSAAPVSSTSSLPLAALNMMAKNTITKTLKLRIVRPYNSAEVEKIVADEKNNREKIALEKNKDKVKEACSKHLKVAAYCTTQVERNACLFCKARKLDDKFYQKLRGQFPDAVFWQEISEIFRQLQKQAAEIYNQSLIELYYEIFIKGKGIANASSVEHYLSDVCYTRAAELFKNAAIASGLRSKIKSNFRLKELKNMKSGLPTTKSDNFPIPLVKQKGGQYTGFEISNHNSDFIIKIPFGRWQVKKEIDKYRPWEKFDFEQVQKSPKPISLLLSTQRRKRNKGWSKDEGTEAEIKKVMNGDYQTSYIEVKRGSKIGEKSAWMLNLSIDVPKIDKGVDPSIIGGIDVGVKSPLVCAINNAFSRYSISDNDLFHFNKKMFARRRILLKKNRHKRAGHGAKNKLKPITILTEKSERFRKKLIERWACEIADFFIKNKVGTVQMENLESMKRKEDSYFNIRLRGFWPYAEMQNKIEFKLKQYGIEIRKVAPNNTSKTCSKCGHLNNYFNFEYRKKNKFPHFKCEKCNFKENADYNAALNISNPKLKSTKEEP

SEQ ID NO: 292 - RNA, 140 nt, Artificial Sequence; identical to SEQ ID NO: 112
  tracrRNA scaffold of Cas12f1, MF

SEQ ID NO: 293 - RNA, 32 nt, Artificial Sequence
  1st Fragment of engineered tracrRNA scaffold
caaauucannncnccucuccaauucugcacaa

SEQ ID NO: 294 - RNA, 31 nt, Artificial Sequence
  1st Fragment of engineered tracrRNA scaffold
caaauucannncnccucuccaauucugcaca

SEQ ID NO: 295 - RNA, 30 nt, Artificial Sequence
  1st Fragment of engineered tracrRNA scaffold
caaauucannncnccucuccaauucugcac

SEQ ID NO: 296 - RNA, 29 nt, Artificial Sequence
  1st Fragment of engineered tracrRNA scaffold
caaauucannncnccucuccaauucugca

SEQ ID NO: 297 - RNA, 28 nt, Artificial Sequence
  1st Fragment of engineered tracrRNA scaffold
caaauucannncnccucuccaauucugc

SEQ ID NO: 298 - RNA, 27 nt, Artificial Sequence
  1st Fragment of engineered tracrRNA scaffold
caaauucannncnccucuccaauucug

SEQ ID NO: 299 - RNA, 26 nt, Artificial Sequence
  1st Fragment of engineered tracrRNA scaffold
caaauucannncnccucuccaauucu

SEQ ID NO: 300 - RNA, 25 nt, Artificial Sequence
  1st Fragment of engineered tracrRNA scaffold
caaauucannncnccucuccaauuc

SEQ ID NO: 301 - RNA, 24 nt, Artificial Sequence
  1st Fragment of engineered tracrRNA scaffold
caaauucannncnccucuccaauu

SEQ ID NO: 302 - RNA, 23 nt, Artificial Sequence
  1st Fragment of engineered tracrRNA scaffold
caaauucannncnccucuccaau

SEQ ID NO: 303 - RNA, 22 nt, Artificial Sequence
  1st Fragment of engineered tracrRNA scaffold
caaauucannncnccucuccaa

SEQ ID NO: 304 - RNA, 21 nt, Artificial Sequence
  1st Fragment of engineered tracrRNA scaffold
caaauucannncnccucucca

SEQ ID NO: 305 - RNA, 20 nt, Artificial Sequence
  1st Fragment of engineered tracrRNA scaffold
caaauucannncnccucucc

SEQ ID NO: 306 - RNA, 19 nt, Artificial Sequence
  1st Fragment of engineered tracrRNA scaffold
caaauucannncnccucuc

SEQ ID NO: 307 - RNA, 18 nt, Artificial Sequence
  1st Fragment of engineered tracrRNA scaffold
caaauucannncnccucu

SEQ ID NO: 308 - RNA, 17 nt, Artificial Sequence
  1st Fragment of engineered tracrRNA scaffold
caaauucannncnccuc

SEQ ID NO: 309 - RNA, 16 nt, Artificial Sequence
  1st Fragment of engineered tracrRNA scaffold
caaauucannncnccu

SEQ ID NO: 310 - RNA, 15 nt, Artificial Sequence
  1st Fragment of engineered tracrRNA scaffold
caaauucannncncc

SEQ ID NO: 311 - RNA, 14 nt, Artificial Sequence
  1st Fragment of engineered tracrRNA scaffold
caaauucannncnc

SEQ ID NO: 312 - RNA, 13 nt, Artificial Sequence
  1st Fragment of engineered tracrRNA scaffold
caaauucannncn

SEQ ID NO: 313 - RNA, 39 nt, Artificial Sequence
  2nd Fragment of engineered tracrRNA scaffold
augucgagaagugcuuucuucggaaaguaacccucgaaa

SEQ ID NO: 314 - RNA, 19 nt, Artificial Sequence
  3rd Fragment of engineered tracrRNA scaffold
ggcugcuugcaucagccua

SEQ ID NO: 315 - RNA, 50 nt, Artificial Sequence
  4th Fragment of engineered tracrRNA scaffold
ccgcuucaccaaaagcugucccuuaggggauuagaacuugagugaaggug

SEQ ID NO: 316 - RNA, 48 nt, Artificial Sequence
  4th Fragment of engineered tracrRNA scaffold
ccgcuucaccaaaagcuguccuuagggauuagaacuugagugaaggug

SEQ ID NO: 317 - RNA, 46 nt, Artificial Sequence
  4th Fragment of engineered tracrRNA scaffold
ccgcuucaccaaaagcugucuuaggauuagaacuugagugaaggug

SEQ ID NO: 318 - RNA, 44 nt, Artificial Sequence
  4th Fragment of engineered tracrRNA scaffold
ccgcuucaccaaaagcuguuuagauuagaacuugagugaaggug

SEQ ID NO: 319 - RNA, 42 nt, Artificial Sequence
  4th Fragment of engineered tracrRNA scaffold
ccgcuucaccaaaagcuguuaguuagaacuugagugaaggug

SEQ ID NO: 320 - RNA, 41 nt, Artificial Sequence
  4th Fragment of engineered tracrRNA scaffold
ccgcuucaccaaaagcuguuaguagaacuugagugaaggug

SEQ ID NO: 321 - RNA, 39 nt, Artificial Sequence
  4th Fragment of engineered tracrRNA scaffold
ccgcuucaccaaaagcuuuagagaacuugagugaaggug

SEQ ID NO: 322 - RNA, 37 nt, Artificial Sequence
  4th Fragment of engineered tracrRNA scaffold
ccgcuucaccaaaagcuuaggaacuugagugaaggug

SEQ ID NO: 323 - RNA, 35 nt, Artificial Sequence
  4th Fragment of engineered tracrRNA scaffold
ccgcuucaccaaaaguuagaacuugagugaaggug

SEQ ID NO: 324 - RNA, 33 nt, Artificial Sequence
  4th Fragment of engineered tracrRNA scaffold
ccgcuucaccaaaauuagacuugagugaaggug

SEQ ID NO: 325 - RNA, 31 nt, Artificial Sequence
  4th Fragment of engineered tracrRNA scaffold
ccgcuucaccaaauuagcuugagugaaggug

SEQ ID NO: 326 - RNA, 29 nt, Artificial Sequence
  4th Fragment of engineered tracrRNA scaffold
ccgcuucaccaauuaguugagugaaggug

SEQ ID NO: 327 - RNA, 27 nt, Artificial Sequence
  4th Fragment of engineered tracrRNA scaffold
ccgcuucaccauuagugagugaaggug

SEQ ID NO: 328 - RNA, 25 nt, Artificial Sequence
  4th Fragment of engineered tracrRNA scaffold
ccgcuucaccuuaggagugaaggug

SEQ ID NO: 329 - RNA, 23 nt, Artificial Sequence
  4th Fragment of engineered tracrRNA scaffold
ccgcuucacuuagagugaaggug

SEQ ID NO: 330 - RNA, 22 nt, Artificial Sequence
  4th Fragment of engineered tracrRNA scaffold
ccgcuucacuuaggugaaggug

SEQ ID NO: 331 - RNA, 20 nt, Artificial Sequence
  4th Fragment of engineered tracrRNA scaffold
ccgcuucauuagugaaggug

SEQ ID NO: 332 - RNA, 18 nt, Artificial Sequence
  4th Fragment of engineered tracrRNA scaffold
ccgcuucuuaggaaggug

SEQ ID NO: 333 - RNA, 16 nt, Artificial Sequence
  4th Fragment of engineered tracrRNA scaffold
ccgcuuuuagaaggug

SEQ ID NO: 334 - RNA, 14 nt, Artificial Sequence
  4th Fragment of engineered tracrRNA scaffold
ccgcuuuagaggug

SEQ ID NO: 335 - RNA, 12 nt, Artificial Sequence
  4th Fragment of engineered tracrRNA scaffold
ccgcuuagggug

SEQ ID NO: 336 - RNA, 10 nt, Artificial Sequence
  4th Fragment of engineered tracrRNA scaffold
ccguuaggug

SEQ ID NO: 337 - RNA, 21 nt, Artificial Sequence
  5th Fragment of engineered tracrRNA scaffold
cuucacugauaaaguggagaa

SEQ ID NO: 338 - RNA, 10 nt, Artificial Sequence
  5th Fragment of engineered tracrRNA scaffold
aaguggagaa

SEQ ID NO: 339 - RNA, 11 nt, Artificial Sequence
  5th Fragment of engineered tracrRNA scaffold
aaaguggagaa

SEQ ID NO: 340 - RNA, 12 nt, Artificial Sequence
  5th Fragment of engineered tracrRNA scaffold
uaaaguggagaa

SEQ ID NO: 341 - RNA, 13 nt, Artificial Sequence
  5th Fragment of engineered tracrRNA scaffold
auaaaguggagaa

SEQ ID NO: 342 - RNA, 14 nt, Artificial Sequence
  5th Fragment of engineered tracrRNA scaffold
gauaaaguggagaa

SEQ ID NO: 343 - RNA, 15 nt, Artificial Sequence
  5th Fragment of engineered tracrRNA scaffold
ugauaaaguggagaa

SEQ ID NO: 344 - RNA, 16 nt, Artificial Sequence
  5th Fragment of engineered tracrRNA scaffold
cugauaaaguggagaa

SEQ ID NO: 345 - RNA, 17 nt, Artificial Sequence
  5th Fragment of engineered tracrRNA scaffold
acugauaaaguggagaa

SEQ ID NO: 346 - RNA, 18 nt, Artificial Sequence
  5th Fragment of engineered tracrRNA scaffold
cacugauaaaguggagaa

SEQ ID NO: 347 - RNA, 19 nt, Artificial Sequence
  5th Fragment of engineered tracrRNA scaffold
ucacugauaaaguggagaa

SEQ ID NO: 348 - RNA, 20 nt, Artificial Sequence
  5th Fragment of engineered tracrRNA scaffold
uucacugauaaaguggagaa

SEQ ID NO: 349 - RNA, 10 nt, Artificial Sequence
  1st region of engineered tracrRNA scaffold, MF
aaguggagaa

SEQ ID NO: 350 - RNA, 11 nt, Artificial Sequence
  1st region of engineered tracrRNA scaffold, MF
aaaguggagaa

SEQ ID NO: 351 - RNA, 12 nt, Artificial Sequence
  1st region of engineered tracrRNA scaffold, MF
uaaaguggagaa

SEQ ID NO: 352 - RNA, 13 nt, Artificial Sequence
  1st region of engineered tracrRNA scaffold, MF
auaaaguggagaa

SEQ ID NO: 353 - RNA, 14 nt, Artificial Sequence
  1st region of engineered tracrRNA scaffold, MF
gauaaaguggagaa

SEQ ID NO: 354 - RNA, 15 nt, Artificial Sequence
  1st region of engineered tracrRNA scaffold, MF
ugauaaaguggagaa

SEQ ID NO: 355 - RNA, 16 nt, Artificial Sequence
  1st region of engineered tracrRNA scaffold, MF
cugauaaaguggagaa

SEQ ID NO: 356 - RNA, 17 nt, Artificial Sequence
  1st region of engineered tracrRNA scaffold, MF
acugauaaaguggagaa

SEQ ID NO: 357 - RNA, 18 nt, Artificial Sequence
  1st region of engineered tracrRNA scaffold, MF
cacugauaaaguggagaa

SEQ ID NO: 358 - RNA, 19 nt, Artificial Sequence
  1st region of engineered tracrRNA scaffold, MF
ucacugauaaaguggagaa

SEQ ID NO: 359 - RNA, 20 nt, Artificial Sequence
  1st region of engineered tracrRNA scaffold, MF
uucacugauaaaguggagaa

SEQ ID NO: 360 - RNA, 21 nt, Artificial Sequence
  1st region of engineered tracrRNA scaffold, MF
cuucacugauaaaguggagaa

SEQ ID NO: 361 - RNA, 10 nt, Artificial Sequence
  2nd region of engineered tracrRNA scaffold, MF
ccuuaggugg

SEQ ID NO: 362 - RNA, 11 nt, Artificial Sequence
  2nd region of engineered tracrRNA scaffold, MF
ccguuaggugg

SEQ ID NO: 363 - RNA, 13 nt, Artificial Sequence
  2nd region of engineered tracrRNA scaffold, MF
ccgcuuagggugg

SEQ ID NO: 364 - RNA, 15 nt, Artificial Sequence
  2nd region of engineered tracrRNA scaffold, MF
ccgcuuuagaggugg

SEQ ID NO: 365 - RNA, 17 nt, Artificial Sequence
  2nd region of engineered tracrRNA scaffold, MF
ccgcuuuuagaaggugg

SEQ ID NO: 366 - RNA, 19 nt, Artificial Sequence
  2nd region of engineered tracrRNA scaffold, MF
ccgcuucuuaggaaggugg

SEQ ID NO: 367 - RNA, 21 nt, Artificial Sequence
  2nd region of engineered tracrRNA scaffold, MF
ccgcuucauuagugaaggugg

SEQ ID NO: 368 - RNA, 23 nt, Artificial Sequence
  2nd region of engineered tracrRNA scaffold, MF
ccgcuucacuuaggugaaggugg

SEQ ID NO: 369 - RNA, 24 nt, Artificial Sequence
  2nd region of engineered tracrRNA scaffold, MF
ccgcuucacuuagagugaaggugg

SEQ ID NO: 370 - RNA, 26 nt, Artificial Sequence
  2nd region of engineered tracrRNA scaffold, MF
ccgcuucaccuuaggagugaaggugg

SEQ ID NO: 371 - RNA, 28 nt, Artificial Sequence
  2nd region of engineered tracrRNA scaffold, MF
ccgcuucaccauuagugagugaaggugg

SEQ ID NO: 372 - RNA, 30 nt, Artificial Sequence
  2nd region of engineered tracrRNA scaffold, MF
ccgcuucaccaauuaguugagugaaggugg

SEQ ID NO: 373 - RNA, 32 nt, Artificial Sequence
  2nd region of engineered tracrRNA scaffold, MF
ccgcuucaccaaauuagcuugagugaaggugg

SEQ ID NO: 374 - RNA, 34 nt, Artificial Sequence
  2nd region of engineered tracrRNA scaffold, MF
ccgcuucaccaaaauuagacuugagugaaggugg

SEQ ID NO: 375 - RNA, 36 nt, Artificial Sequence
  2nd region of engineered tracrRNA scaffold, MF
ccgcuucaccaaaaguuagaacuugagugaaggugg

SEQ ID NO: 376 - RNA, 38 nt, Artificial Sequence
  2nd region of engineered tracrRNA scaffold, MF
ccgcuucaccaaaagcuuaggaacuugagugaaggugg

SEQ ID NO: 377 - RNA, 40 nt, Artificial Sequence
  2nd region of engineered tracrRNA scaffold, MF
ccgcuucaccaaaagcuuuagagaacuugagugaaggugg

SEQ ID NO: 378 - RNA, 42 nt, Artificial Sequence
  2nd region of engineered tracrRNA scaffold, MF
ccgcuucaccaaaagcuguuaguagaacuugagugaaggugg

SEQ ID NO: 379 - RNA, 43 nt, Artificial Sequence
  2nd region of engineered tracrRNA scaffold, MF
ccgcuucaccaaaagcuguuaguuagaacuugagugaaggugg

SEQ ID NO: 380 - RNA, 45 nt, Artificial Sequence
  2nd region of engineered tracrRNA scaffold, MF
ccgcuucaccaaaagcuguuuagauuagaacuugagugaaggugg

SEQ ID NO: 381 - RNA, 47 nt, Artificial Sequence
  2nd region of engineered tracrRNA scaffold, MF
ccgcuucaccaaaagcugucuuaggauuagaacuugagugaaggugg

SEQ ID NO: 382 - RNA, 51 nt, Artificial Sequence
  2nd region of engineered tracrRNA scaffold, MF
ccgcuucaccaaaagcugucccuuaggggauuagaacuugagugaaggugg

SEQ ID NO: 383 - RNA, 55 nt, Artificial Sequence
  3rd region of engineered tracrRNA scaffold, MF
gcugcuugcaucagccuaaugucgagaagugcuuucuucggaaaguaacccucga

SEQ ID NO: 384 - RNA, 53 nt, Artificial Sequence
  3rd region of engineered tracrRNA scaffold, MF
gcugcuugcaucagccuaaugucgagaagugcuuuuucgaaaguaacccucga

SEQ ID NO: 385 - RNA, 51 nt, Artificial Sequence
  3rd region of engineered tracrRNA scaffold, MF
gcugcuugcaucagccuaaugucgagaagugcuuuucgaaguaacccucga

SEQ ID NO: 386 - RNA, 51 nt, Artificial Sequence
  3rd region of engineered tracrRNA scaffold, MF
gcugcuugcaucagccuaaugucgagaagugcucuucggaguaacccucga

SEQ ID NO: 387 - RNA, 49 nt, Artificial Sequence
  3rd region of engineered tracrRNA scaffold, MF
gcugcuugcaucagccuaaugucgagaagugcuuucgaguaacccucga

SEQ ID NO: 388 - RNA, 47 nt, Artificial Sequence
  3rd region of engineered tracrRNA scaffold, MF
gcugcuugcaucagccuaaugucgagaagugcuucgguaacccucga

SEQ ID NO: 389 - RNA, 45 nt, Artificial Sequence
  3rd region of engineered tracrRNA scaffold, MF
gcugcuugcaucagccuaaugucgagaaguguucguaacccucga

SEQ ID NO: 390 - RNA, 43 nt, Artificial Sequence
  3rd region of engineered tracrRNA scaffold, MF
gcugcuugcaucagccuaaugucgagaaguuucgaacccucga

SEQ ID NO: 391 - RNA, 41 nt, Artificial Sequence
  3rd region of engineered tracrRNA scaffold, MF
gcugcuugcaucagccuaaugucgagaaguucgacccucga

SEQ ID NO: 392 - RNA, 40 nt, Artificial Sequence
  3rd region of engineered tracrRNA scaffold, MF
gcugcuugcaucagccuaaugucgagaaguucgcccucga

SEQ ID NO: 393 - RNA, 39 nt, Artificial Sequence
  3rd region of engineered tracrRNA scaffold, MF
gcugcuugcaucagccuaaugucgagaauucgcccucga

SEQ ID NO: 394 - RNA, 38 nt, Artificial Sequence
  3rd region of engineered tracrRNA scaffold, MF
gcugcuugcaucagccuaaugucgagaauucgccucga

SEQ ID NO: 395 - RNA, 37 nt, Artificial Sequence
  3rd region of engineered tracrRNA scaffold, MF
gcugcuugcaucagccuaaugucgagauucgccucga

SEQ ID NO: 396 - RNA, 35 nt, Artificial Sequence
  3rd region of engineered tracrRNA scaffold, MF
gcugcuugcaucagccuaaugucgaguucgcucga

SEQ ID NO: 397 - RNA, 55 nt, Artificial Sequence; identical to SEQ ID NO: 383
  3rd region of engineered tracrRNA scaffold, MF

SEQ ID NO: 398 - RNA, 6 nt, Artificial Sequence
  4th region of engineered tracrRNA scaffold, MF
aacaaa

SEQ ID NO: 399 - RNA, 7 nt, Artificial Sequence
  4th region of engineered tracrRNA scaffold, MF
aacaaau

SEQ ID NO: 400 - RNA, 8 nt, Artificial Sequence
  4th region of engineered tracrRNA scaffold, MF
aacaaauu

SEQ ID NO: 401 - RNA, 9 nt, Artificial Sequence
  4th region of engineered tracrRNA scaffold, MF
aacaaauuc

SEQ ID NO: 402 - RNA, 10 nt, Artificial Sequence
  4th region of engineered tracrRNA scaffold, MF
aacaaauuca

SEQ ID NO: 403 - RNA, 11 nt, Artificial Sequence
  4th region of engineered tracrRNA scaffold, MF
aacaaauucau

SEQ ID NO: 404 - RNA, 12 nt, Artificial Sequence
  4th region of engineered tracrRNA scaffold, MF
aacaaauucauu

SEQ ID NO: 405 - RNA, 13 nt, Artificial Sequence
  4th region of engineered tracrRNA scaffold, MF
aacaaauucauuu

SEQ ID NO: 406 - RNA, 17 nt, Artificial Sequence
  crRNA scaffold of Cas12f1, MF
gaaugaaggaaugcaac

SEQ ID NO: 407 - RNA, 30 nt, Artificial Sequence
  6th fragment of engineered crRNA scaffold, WT
guugcagaacccgaauagnbnnnugaagga

SEQ ID NO: 408 - RNA, 30 nt, Artificial Sequence
  6th fragment of engineered crRNA scaffold, WT
guugcagaacccgaauagngnnnugaagga

SEQ ID NO: 409 - RNA, 29 nt, Artificial Sequence
  6th fragment of engineered crRNA scaffold, WT
uugcagaacccgaauagngnnnugaagga

SEQ ID NO: 410 - RNA, 28 nt, Artificial Sequence
  6th fragment of engineered crRNA scaffold, WT
ugcagaacccgaauagngnnnugaagga

SEQ ID NO: 411 - RNA, 27 nt, Artificial Sequence
  6th fragment of engineered crRNA scaffold, WT
gcagaacccgaauagngnnnugaagga

SEQ ID NO: 412 - RNA, 26 nt, Artificial Sequence
  6th fragment of engineered crRNA scaffold, WT
cagaacccgaauagngnnnugaagga

SEQ ID NO: 413 - RNA, 25 nt, Artificial Sequence
  6th fragment of engineered crRNA scaffold, WT
agaacccgaauagngnnnugaagga

SEQ ID NO: 414 - RNA, 24 nt, Artificial Sequence
  6th fragment of engineered crRNA scaffold, WT
gaacccgaauagngnnnugaagga

SEQ ID NO: 415 - RNA, 23 nt, Artificial Sequence
  6th fragment of engineered crRNA scaffold, WT
aacccgaauagngnnnugaagga

SEQ ID NO: 416 - RNA, 22 nt, Artificial Sequence
  6th fragment of engineered crRNA scaffold, WT
acccgaauagngnnnugaagga

SEQ ID NO: 417 - RNA, 21 nt, Artificial Sequence
  6th fragment of engineered crRNA scaffold, WT
cccgaauagngnnnugaagga

SEQ ID NO: 418 - RNA, 20 nt, Artificial Sequence
  6th fragment of engineered crRNA scaffold, WT
ccgaauagngnnnugaagga

SEQ ID NO: 419 - RNA, 19 nt, Artificial Sequence
  6th fragment of engineered crRNA scaffold, WT
cgaauagngnnnugaagga

SEQ ID NO: 420 - RNA, 18 nt, Artificial Sequence
  6th fragment of engineered crRNA scaffold, WT
gaauagngnnnugaagga

SEQ ID NO: 421 - RNA, 17 nt, Artificial Sequence
  6th fragment of engineered crRNA scaffold, WT
aauagngnnnugaagga

SEQ ID NO: 422 - RNA, 16 nt, Artificial Sequence
  6th fragment of engineered crRNA scaffold, WT
auagngnnnugaagga

SEQ ID NO: 423 - RNA, 15 nt, Artificial Sequence
  6th fragment of engineered crRNA scaffold, WT
uagngnnnugaagga

SEQ ID NO: 424 - RNA, 14 nt, Artificial Sequence
  6th fragment of engineered crRNA scaffold, WT
agngnnnugaagga

SEQ ID NO: 425 - RNA, 12 nt, Artificial Sequence
  6th fragment of engineered crRNA scaffold, WT
ngnnnugaagga

SEQ ID NO: 426 - RNA, 10 nt, Artificial Sequence
  5th region of engineered crRNA scaffold, MF
gaaugaagga

SEQ ID NO: 427 - RNA, 11 nt, Artificial Sequence
  5th region of engineered crRNA scaffold, MF
cgaaugaagga

SEQ ID NO: 428 - RNA, 12 nt, Artificial Sequence
  5th region of engineered crRNA scaffold, MF
acgaaugaagga

SEQ ID NO: 429 - RNA, 13 nt, Artificial Sequence
  5th region of engineered crRNA scaffold, MF
gacgaaugaagga

SEQ ID NO: 430 - RNA, 14 nt, Artificial Sequence
  5th region of engineered crRNA scaffold, MF
agacgaaugaagga

SEQ ID NO: 431 - RNA, 15 nt, Artificial Sequence
  5th region of engineered crRNA scaffold, MF
uagacgaaugaagga

SEQ ID NO: 432 - RNA, 16 nt, Artificial Sequence
  5th region of engineered crRNA scaffold, MF
auagacgaaugaagga

SEQ ID NO: 433 - RNA, 17 nt, Artificial Sequence
  5th region of engineered crRNA scaffold, MF
aauagacgaaugaagga

SEQ ID NO: 434 - RNA, 18 nt, Artificial Sequence
  5th region of engineered crRNA scaffold, MF
gaauagacgaaugaagga

SEQ ID NO: 435 - RNA, 19 nt, Artificial Sequence
  5th region of engineered crRNA scaffold, MF
cgaauagacgaaugaagga

SEQ ID NO: 436 - RNA, 20 nt, Artificial Sequence
  5th region of engineered crRNA scaffold, MF
ccgaauagacgaaugaagga

SEQ ID NO: 437 - RNA, 21 nt, Artificial Sequence
  5th region of engineered crRNA scaffold, MF
cccgaauagacgaaugaagga

SEQ ID NO: 438 - RNA, 22 nt, Artificial Sequence
  5th region of engineered crRNA scaffold, MF
acccgaauagacgaaugaagga

SEQ ID NO: 439 - RNA, 23 nt, Artificial Sequence
  5th region of engineered crRNA scaffold, MF
aacccgaauagacgaaugaagga

SEQ ID NO: 440 - RNA, 24 nt, Artificial Sequence
  5th region of engineered crRNA scaffold, MF
gaacccgaauagacgaaugaagga

SEQ ID NO: 441 - RNA, 25 nt, Artificial Sequence
  5th region of engineered crRNA scaffold, MF
agaacccgaauagacgaaugaagga

SEQ ID NO: 442 - RNA, 26 nt, Artificial Sequence
  5th region of engineered crRNA scaffold, MF
cagaacccgaauagacgaaugaagga

SEQ ID NO: 443 - RNA, 27 nt, Artificial Sequence
  5th region of engineered crRNA scaffold, MF
gcagaacccgaauagacgaaugaagga

SEQ ID NO: 444 - RNA, 28 nt, Artificial Sequence
  5th region of engineered crRNA scaffold, MF
ugcagaacccgaauagacgaaugaagga

SEQ ID NO: 445 - RNA, 29 nt, Artificial Sequence
  5th region of engineered crRNA scaffold, MF
uugcagaacccgaauagacgaaugaagga

SEQ ID NO: 446 - RNA, 47 nt, Artificial Sequence
  shRNA sequence targeting ATM1
ggagccagauaguuuguauuucaagagaauacaaacuaucuggcucc

SEQ ID NO: 447 - RNA, 47 nt, Artificial Sequence
  shRNA sequence targeting ATM1
gcaagcagcugaaacaaauuucaagagaauuuguuucagcugcuugc

SEQ ID NO: 448 - RNA, 47 nt, Artificial Sequence
  shRNA sequence targeting ATM1
ggagcugauuguagcaacauucaagagauguugcuacaaucagcucc

SEQ ID NO: 449 - RNA, 47 nt, Artificial Sequence
  shRNA sequence targeting ATM1
gcacagaagugccuccaauuucaagagaauuggaggcacuucugugc

SEQ ID NO: 450 - RNA, 47 nt, Artificial Sequence
  shRNA sequence targeting ATM1
ggacauaguuucugggagauucaagagaucucccagaaacuaugucc

SEQ ID NO: 451 - RNA, 47 nt, Artificial Sequence
  shRNA sequence targeting XRCC4
ggaugacacuggcacauuauucaagagauaaugugccagugucaucc

SEQ ID NO: 452 - RNA, 47 nt, Artificial Sequence
  shRNA sequence targeting XRCC4
ggagaguacugaugaggaauucaagagauuccucaucaguacucucc

SEQ ID NO: 453 - RNA, 47 nt, Artificial Sequence
  shRNA sequence targeting XRCC4
gaauccaccuuguuucugauucaagagaucagaaacaagguggauuc

SEQ ID NO: 454 - RNA, 47 nt, Artificial Sequence
  shRNA sequence targeting XRCC4
guacaaguaucuugggagauucaagagaucucccaagauacuuguac

SEQ ID NO: 455 - RNA, 47 nt, Artificial Sequence
  shRNA sequence targeting XRCC4
gaaugcagcucaagaacgauucaagagaucguucuugagcugcauuc

SEQ ID NO: 456 - RNA, 47 nt, Artificial Sequence
  shRNA sequence targeting XLF-1
gcaugagucuggcauuacauucaagagauguaaugccagacucaugc

SEQ ID NO: 457 - RNA, 47 nt, Artificial Sequence
  shRNA sequence targeting XLF-1
gaaagcccuuugucaugaauucaagagauucaugacaaagggcuuuc

SEQ ID NO: 458 - RNA, 47 nt, Artificial Sequence
  shRNA sequence targeting XLF-1
gaacagugcuucccugcaauucaagagauugcagggaagcacuguuc

SEQ ID NO: 459 - RNA, 47 nt, Artificial Sequence
  shRNA sequence targeting XLF-1
ggaaagaccuagagauccauucaagagauggaucucuaggucuuucc

SEQ ID NO: 460 - RNA, 47 nt, Artificial Sequence
  shRNA sequence targeting XLF-1
guauggcagucaccacacauucaagagauguguggugacugccauac

SEQ ID NO: 461 - RNA, 47 nt, Artificial Sequence
  shRNA sequence targeting XRCC6
gcagcauugugcagauacauucaagagauguaucugcacaaugcugc

SEQ ID NO: 462 - RNA, 47 nt, Artificial Sequence
  shRNA sequence targeting XRCC6
gcaggaacaucccuccuuauucaagagauaaggagggauguuccugc

SEQ ID NO: 463 - RNA, 47 nt, Artificial Sequence
  shRNA sequence targeting XRCC6
gcagugcucugcucaucaauucaagagauugaugagcagagcacugc

SEQ ID NO: 464 - RNA, 47 nt, Artificial Sequence
  shRNA sequence targeting XRCC6
ggaucaugcuguucaccaauucaagagauuggugaacagcaugaucc

SEQ ID NO: 465 - RNA, 47 nt, Artificial Sequence
  shRNA sequence targeting XRCC6
ggaucugacuacucacucauucaagagaugagugaguagucagaucc

SEQ ID NO: 466 - RNA, 47 nt, Artificial Sequence
  shRNA sequence targeting LIG4
gcacaaagauggagauguauucaagagauacaucuccaucuuugugc

SEQ ID NO: 467 - RNA, 47 nt, Artificial Sequence
  shRNA sequence targeting LIG4
gcagacacguacuguguaauucaagagauuacacaguacgugucugc

SEQ ID NO: 468 - RNA, 47 nt, Artificial Sequence
  shRNA sequence targeting LIG4
ggagcagacuccugaagaauucaagagauucuucaggagucugcucc

SEQ ID NO: 469 - RNA, 47 nt, Artificial Sequence
  shRNA sequence targeting LIG4
ggaggauucugaucugcaauucaagagauugcagaucagaauccucc

SEQ ID NO: 470 - RNA, 47 nt, Artificial Sequence
  shRNA sequence targeting LIG4
gcaugauccuucuguaggauucaagagauccuacagaaggaucaugc

SEQ ID NO: 471 - RNA, 47 nt, Artificial Sequence
  shRNA sequence targeting DCLRE1C
ggagacuccuacccagauauucaagagauaucuggguaggagucucc

SEQ ID NO: 472 - RNA, 47 nt, Artificial Sequence
  shRNA sequence targeting DCLRE1C
ggacaaagcugacuacagauucaagagaucuguagucagcuuugucc

SEQ ID NO: 473 - RNA, 47 nt, Artificial Sequence
  shRNA sequence targeting DCLRE1C
gcagagcucucguuucacauucaagagaugugaaacgagagcucugc

SEQ ID NO: 474 - RNA, 47 nt, Artificial Sequence
  shRNA sequence targeting DCLRE1C
ggacucugauggagaaucauucaagagaugauucuccaucagagucc

SEQ ID NO: 475 - RNA, 47 nt, Artificial Sequence
  shRNA sequence targeting DCLRE1C
gcagaauucuucccagucauucaagagaugacugggaagaauucugc

SEQ ID NO: 476 - RNA, 8192 nt, Artificial Sequence
  661W/LCA10 cell line doner sequence
tctagacctaacatacatactacttctgctcggttataaagtaatctaattccttaaggagccctatttctttgtagagatgaaaatatttccatgcccagaacttattacaccatgtctgtcattgctttgagaatattattgctgcttctctctttccttggacaacatgtaatgtatatctttagaatgtgaattcatatttaactttgtagttttatgttcttcactattttacatacagctgagagattaaagtatttatatcatatattaatttaaaataataacagctgtaatacttcttaatatatcctaaaaccgctttaaagttcttatgttccttggaatctatctcctgaacatacattggcaaaaataacatattctagtaatttgaaatgatactttttgctttcaatattaggattttttttttgagctgaaatgaactatataaaacatttgtattttcaaaagattcagtgtgaagtgtctagctgctgcccctgccctgctaccctgataacagaatatcctccaggtagctcttctgcaacagaagcagtcacgtgcatctggactgtcacgtgagagctggctctctcagatgaggaagttttgagacttacaaatgttcttgtttttattattgtggcttttaaaacatattggacttttctgaagttttgccagtacagagagtatgaaatatacgagctggaggtttctgccatcctccttctttcttgtttcttcaaccacagtttttagggttcgtgatttttttcttttttatagaaaataagaaaagaggatattttaacggaaacaagacataattcatgtcttttaaccagccttcactgcaaaatgaaaccagatgcctctaaggtagaatagtatatgctcatttacatgaggggaagctgtttgaattagacagaaagttcactacactcaggagtgaattagaactataagagcctcatctccccttcagtggtttggttctttgttgctcccatgatctcactgtactttcttatcatggagcatttcactgggaagaactggaaagagtcccggctccttgttggtgttcatcaaaccacctcctgccattcatgaatgccttttcagagctatcggagaatattgcgttaccctcttcccaggactctaccgaatacctcagattattaaacttagaaacagaaaaaggttgttttggttcagctacttgaaggtttgggactatgacctcattacctttggactgtggtaactcgtatacatcatagtaagagggcgggtaatagggaccttgtcacttcatagccaattataatgaaaagaaaaagagggcaccaagacaaaggtcccacggtcctctttgaaagcacaactaaagtgatcttagagttcacaccagcaccagtcttagctggtgccacttccggattgcaccgtgccggagaagactgtagcatgtgtctttgggggaatgttctatattaaactatagcaaacatgaaataagtcaattaaatccttattgttactatttaggtattttaatcagtcgataacaagaaccaaaccttgcgtttgtgtcacttgaagaaagcagacatagacagcatacattaattctgtcacttaaactgccagatgcttagtggattttaatcttctatgacttagagaaggtatccaaagatatcttctgcttactatactttctcaaattcattgtacttcctttttctctgataacttgtaaaaggactcacttaaatccttaattaaaactttccaaataattgttttctacgagaaagaataacaggaaatattacacatttttcaaatggctttcaactattttgctttcaattgaattttctttttaaaaagtgactaaggctttgccagaaaaaaatatgcaaagttaacttggtatatcctttttttttttttttttttttatttttcaggaaatggccattttcaagattgcagctctccaaaaagttgtagataatagtgtttctttgtctgaactagaactggctaataaacagtacaatgaactgactgctaagtacagggacatcttgcaaaaagataatatgcttgttcaaagaacaagtaacttggaacacctggaggtaagtttgtgtgattcttgaaccttgtgaaattagccatttttcttcaatatttttgtgtttggggggatttggcagattttaattaaagtttgcctgcatttatataaatttaacagagatataattatccatattattcattcagtttagttataaatattttgttcccacataacacacacacacacacacaatatattatctatttatagtggctgaatgacttctgaatgattatctagatcattctccttaggtcacttgcatgatttagctgaatcaaacctcttttaaccagacatctaagagaaaaaggagcatgaaacaggtagaatattgtaatcaaaggagggaagcactcattaagtgcccatccctttctcttacccctgtacccagaacaaactattctcccatggtccctggcttttgttccttggaatggatgtagccaacagtagctgaaatattaagggctcttcctggaccatggatgcactctgtaaattctcatcattttttattgtagaataaatgtagaattttaatgtagaataaatttatttaatgtagaataaaaaataaaaaaactagagtagaatatcataagttacaatctgtgaatatggaccagaccctttgtagttatcttacagccacttgaactctataccttttactgaggacagaacaagctcctgattttttcatcttcctcatcagaaatagaggcttatggattttggattattcttatctaagatcctttcacaggagtagaataagatctaattctattagctcaaaagcttttgctggctcatagagacacattcagtaaatgaaaacgttgttctgagtagctttcaggattcctactaaattatgagtcatgtttatcaatattatttagaagtaatcataatcagtttgctttctgctgcttttgccaaagagaggtgattatgttactttttatagaaaattatgcctatttagtgtggtgataatttatttttttccattctccatgtcctctgtcctatcctctccagcattagaaagtcctaggcaagagacatcttgtggataatgtatcaatgagtgatgtttaacgttatcattttcccaaagagtatttttcatctttcctaaagattttttttttttttgagatggagtttcattctgtcacccaggctgagtgcagtggcacgatctcggcttaacgcttactgcatcctctgcctcccagattcaagcagttctcctgcctcagcctctgagtagctgggattacaggtgtgcaccaccacagcagctaatttttttttttttttttttttttttgaggcagagtctcgctctgtcacccaggctggagtgcagtggcgccatcttggctcactgcaagctccacctcccgggttcaggccgttctcctgcctcagcctcctgagtagctggtaccacaggcacccaccatcatgcccggctaattttttgtatttttagtagagatggggtttcaccttgttagccaggatggtgtcgatctcctgaactcgtgatccacccgcctcggcctcctaaagtgctgggattacagatgtgagccaccgcacctggccccagttgtaattgtgagtatctcatacctatccctattggcagtgtcttagttttattttttattatctttattgtggcagccattattcctgtctctatctccagtcttacatcctccttactgccacaagaatgatcattctaaacatgaatcctaccctgtgactcccatgtgactccccgccttaaaaactgtcaaaagctaccggttacctgaagggtaaaagtcaagtcccctacttacctcatgtcatctaaagcaagagatgaactagctgagttttctgaccacagtgttctttcttatgtatgttcttttgtacgtgctcttttctatatatagggaaccatttctctcttccagttgttttgctcagtgaatttctattcctgtttcaaaacttgttcaggcattaccttttttttcttaagcatactttttttaatggaacaaagtcactcctgtctacactagttctgcatcttatacataggttttgtacatagtacatatttatatcacatcaaattatatgtgtttacatatctgtcttccttaatggaatataagtcttttgatataaggaactatttaatttgtttctgtgtgttgagtatctcctgtttggcacagagttcaagctaatacatgagagtgattagtggtggagagccacagtgcatgtggtgtcaaatatggtgcttaggaaattattgttgctttttgagaggtaaaggttcatgagactagaggtcacgaaaatcagatttcatgtgtgaagaatggaatagataataaggaaatacaaaaactggatgggtaataaagcaaaagaaaaacttgaaatttgatagtagaagaaaaaagaaatagatgtagattgaggtagaatcaagaagaggattctttttttgttgtttttttttttgaaacagagtctcactgtgttgcccaggctggagtgcagtggagtgatcttggcttactgcaacctctgcctcccaggttcaagcgattcttctgcttcagtctcccgagtagctggaattacaggtgcccaccagcacggccggctaatttagtagagacagggttttgccatgttggccgggctggtctcaaactttggatctcaggtaatccgccagcctcaacttcccaaagtgctgggattacaggcatgagccactgtgcccagcctgttttttttttttaaaggagaccagtgaagtttcaggaggagggaaagaaaatttagagttactagggagagagtgatgaagataagagatgaaagtggtaataagggaaatagcaaaatatcagggtaggtgggagaaaaagagatttgtaacaaacaataggattatcctgtgaaaaaggatgaaaggaagaaaaaaatggatagaaagatatttaaaacaccctcagcctcctgttttccctcctgtgtattcatagtatataaaactataattatgtactttacttaaaaaatatattattattaccttatcgtgcttatttaatcatagcatgtcctctttttagtctcattaccctgtttgtattattcttcataacacttaatacctgacattgtattatatattggcttattttccaggtactccactcaaatataagttctaggatataatttatttatcactgaaatccattgcttagagtacctggcatgtagtaaataggcattctgttttttcaaataaaaaataaaggaacttaagatatatatttatgttatatcgccagcctttttcctcacagctctattctgttgtacagaattacctactttacaattcctgtgtttcaaggggatctcaaatttaacgtgtccacaatgaactcctgatttctgtttctctcctagtcattcttatttcaatatatgttcagttacctaaccagctagtcaaggcagatactttagagttattctgtagtcattctttttccctaccatttttgttttccaaatgtaatttatgtgtgtcttcttcatcctcgcagctctaacccttgtccaaaccagcatcatcactcatctggagttccacaatgtctttctggctagtttccctgatttctctattgacccctttattctccacagtgcagccagaatgattgtttaaaacttcctccttaaaatctttaaattgttttcttttatacgttaagttaaattccagttccttgtcttggcatgccatgccctgcctggtgtggcccctgatggtctctccaacttcatgttttactactattgactcttatttttgcttactctgcttgggtgctccagtcctccaaatcatttcctgctccaatcatttcaatcattttttcctctcagatcttatagtattccaaatgctttcttcctttggagcatctgggtttactaataaatacttcgtacctcacagttcagcttaaatatcaattatttggtggttaagacatccttcaaccgctctatctaaatgttcctttctattattcactggctcagtactctgtttttattttctttctaaatgtcaacttttttttttttgagtcagggtctcactgttgcccaggctcgagtgcagttgcacaatcatagctcattgcagccttgccctcctgggatcaagtaattctcccacctcagcctccaaaatagctgggattacaggtatgcatcaccatgctcagctaattttttgtgtttttttgtagagatgaggtctcactttgttgcccaggctggtctcaaactcctggactcaagtgattctcccacctcagcctcccaaagtgctggggttacaggtgtgagccactgcacctggtcgatactgacttttttttttttgagatggagttttgctctgttgcccaggctagagcgcagtggtgtgatctcagctcactgcaacctccacctcccaggttaaagggattcttctgcctcagtctcctgagtagctgggattacaggcaagtgccatcatgactggctaatttttgtatttttagcactatgtttagtactgtgttggccaggcttgtctcgaactcctgacctcaagtgatccacccacctcagcctcccaaagtgctgggattacaggtgtgagccaccgtaatcggccaacattgacatttttagtagactttttgtttgtttacttgcttattatctgctgccttccacactctggcgaaatcctgccacccacccacacacacataggcactgaatgggcagaactctgaaggccagaattttatatttcttttcactataaacatcatcatctgtcactgatggcacactaggatgctcagcaactgtgtgcatgaaggaagtaagcactagtttgtgaaggctgcaaaactcttgagtattctaagagttttggccaaaatgaatgtacagctttagtggcagaagctaatactcagaaattgaggccgtatattggataacacaggatttggatgattattttaaaataatattttacattgtatatatgtgtgtgtgtgtgtgtgtgtgtgtgtgtatgtgtgtgtgtgtgtatatatatatgtatgtatgtgtattagtccgttctcatgctgctatgaagaaatacctgagactgggtaatttataaaggaaagaggtttaattgactcacagttccacagagctggggaggcctcagaaaacttaacagttatggcagaaggggaagcaaacacatttttcttcacatggtggccggaattagaagaatgtgagccgagcaaaggggaaagccccttataaaaccatcagacatcgtgagaacttactattatgagaatagcgtgggggaaaccacccccacgattcaattacctcccaccaaatccctcccatgacatatgaggattatgggaactatgattcaagatgagatttgggtagggacacagccaaaccatatcagtatgtatatgtatacaagtattatatatatatgtatgtgtttgtatgcatacatgtattatatatggaggaaattctaattttgtaaaaaactggattgtgagttttaagataacttcgtatagcatacattatacgaagttataattaaggagcgtgatgcggttttggcagtacatcaatgggcgtggatagcggtttgactcacggggatttccaagtctccaccccattgacgtcaatgggagtttgttttggcaccaaaatcaacgggactttccaaaatgtcgtaacaactccgccccattgacgcaaatgggcggtaggcgtgtacggtgggaggtctatataagcagagctggatgaggatcgtttcgcatgattgaac

SEQ ID NO: 477 - RNA, 127 nt, Artificial Sequence
  guide RNA scaffold sequence (V4.0)
accgcttcaccaaaagctgtcccttaggggattagaacttgagtgaaggtgggctgcttgcatcagcctaatgtcgagaagtgctttcttcggaaagtaaccctcgaaacaaagaaaggaatgcaac

SEQ ID NO: 478 - RNA, 98 nt, Artificial Sequence
  guide RNA scaffold sequence (V4.1)
accgcuucaccgagugaaggugggcugcuugcaucagccuaaugucgagaagugcuuucuucggaaaguaacccucgaaacaaagaaaggaaugcaac

SEQ ID NO: 479 - DNA, 1719 bp, Artificial Sequence
  TnpB Encoding DNA
atgggggagaaaagttcccgccgccgacggaatggaaaaagcggtgcgtggactgctgctataacaagctgtgttgggggtaagatggccaagaacacaattacaaagacactgaagctgaggatcgtgagaccatacaacagcgctgaggtcgagaagattgtggctgatgaaaagaacaacagggaaaagatcgccctcgagaagaacaaggataaggtgaaggaggcctgctctaagcacctgaaagtggccgcctactgcaccacacaggtggagaggaacgcctgtctgttttgtaaagctcggaagctggatgataagttttaccagaagctgcggggccagttccccgatgccgtcttttggcaggagattagcgagatcttcagacagctgcagaagcaggccgccgagatctacaaccagagcctgatcgagctctactacgagatcttcatcaagggcaagggcattgccaacgcctcctccgtggagcactacctgagcgacgtgtgctacacaagagccgccgagctctttaagaacgccgctatcgcttccgggctgaggagcaagattaagagtaacttccggctcaaggagctgaagaacatgaagagcggcctgcccactacaaagagcgacaacttcccaattccactggtgaagcagaaggggggccagtacacagggttcgagatttccaaccacaacagcgactttattattaagatcccctttggcaggtggcaggtcaagaaggagattgacaagtacaggccctgggagaagtttgatttcgagcaggtgcagaagagccccaagcctatttccctgctgctgtccacacagcggcggaagaggaacaaggggtggtctaaggatgaggggaccgaggccgagattaagaaagtgatgaacggcgactaccagacaagctacatcgaggtcaagcggggcagtaagattggcgagaagagcgcctggatgctgaacctgagcattgacgtgccaaagattgataagggcgtggatcccagcatcatcggagggatcgatgtgggggtcaagagccccctcgtgtgcgccatcaacaacgccttcagcaggtacagcatctccgataacgacctgttccactttaacaagaagatgttcgcccggcggaggattttgctcaagaagaaccggcacaagcgggccggacacggggccaagaacaagctcaagcccatcactatcctgaccgagaagagcgagaggttcaggaagaagctcatcgagagatgggcctgcgagatcgccgatttctttattaagaacaaggtcggaacagtgcagatggagaacctcgagagcatgaagaggaaggaggattcctacttcaacattcggctgagggggttctggccctacgctgagatgcagaacaagattgagtttaagctgaagcagtacgggattgagatccggaaggtggcccccaacaacaccagcaagacctgcagcaagtgcgggcacctcaacaactacttcaacttcgagtaccggaagaagaacaagttcccacacttcaagtgcgagaagtgcaactttaaggagaacgccgattacaacgccgccctgaacatcagcaaccctaagctgaagagcactaaggaggagcccaaaaggccggcggccacgaaaaaggccggccaggcaaaaaagaaaaag

SEQ ID NO: 480 - DNA, 1665 bp, Artificial Sequence
  Cas12f1 + CasX 28aa Encoding DNA
atggaaaagagaatcaacaagatcaggaagaagctgagcgccgacaacgccaccaagcctgtgtcaggagtggcccccatggccaagaacacaattacaaagacactgaagctgaggatcgtgagaccatacaacagcgctgaggtcgagaagattgtggctgatgaaaagaacaacagggaaaagatcgccctcgagaagaacaaggataaggtgaaggaggcctgctctaagcacctgaaagtggccgcctactgcaccacacaggtggagaggaacgcctgtctgttttgtaaagctcggaagctggatgataagttttaccagaagctgcggggccagttccccgatgccgtcttttggcaggagattagcgagatcttcagacagctgcagaagcaggccgccgagatctacaaccagagcctgatcgagctctactacgagatcttcatcaagggcaagggcattgccaacgcctcctccgtggagcactacctgagcgacgtgtgctacacaagagccgccgagctctttaagaacgccgctatcgcttccgggctgaggagcaagattaagagtaacttccggctcaaggagctgaagaacatgaagagcggcctgcccactacaaagagcgacaacttcccaattccactggtgaagcagaaggggggccagtacacagggttcgagatttccaaccacaacagcgactttattattaagatcccctttggcaggtggcaggtcaagaaggagattgacaagtacaggccctgggagaagtttgatttcgagcaggtgcagaagagccccaagcctatttccctgctgctgtccacacagcggcggaagaggaacaaggggtggtctaaggatgaggggaccgaggccgagattaagaaagtgatgaacggcgactaccagacaagctacatcgaggtcaagcggggcagtaagattggcgagaagagcgcctggatgctgaacctgagcattgacgtgccaaagattgataagggcgtggatcccagcatcatcggagggatcgatgtgggggtcaagagccccctcgtgtgcgccatcaacaacgccttcagcaggtacagcatctccgataacgacctgttccactttaacaagaagatgttcgcccggcggaggattttgctcaagaagaaccggcacaagcgggccggacacggggccaagaacaagctcaagcccatcactatcctgaccgagaagagcgagaggttcaggaagaagctcatcgagagatgggcctgcgagatcgccgatttctttattaagaacaaggtcggaacagtgcagatggagaacctcgagagcatgaagaggaaggaggattcctacttcaacattcggctgagggggttctggccctacgctgagatgcagaacaagattgagtttaagctgaagcagtacgggattgagatccggaaggtggcccccaacaacaccagcaagacctgcagcaagtgcgggcacctcaacaactacttcaacttcgagtaccggaagaagaacaagttcccacacttcaagtgcgagaagtgcaactttaaggagaacgccgattacaacgccgccctgaacatcagcaaccctaagctgaagagcactaaggaggagccc

SEQ ID NO: 481 - DNA, 1671 bp, Artificial Sequence
  Cas12f1 + random 28aa Encoding DNA
atggctggcggaccaggcgcaggtagtgctgcgccagtttcttcaacttcctccctgcccctggctgcgcttaacatgcgcgtgatggccaagaacacaattacaaagacactgaagctgaggatcgtgagaccatacaacagcgctgaggtcgagaagattgtggctgatgaaaagaacaacagggaaaagatcgccctcgagaagaacaaggataaggtgaaggaggcctgctctaagcacctgaaagtggccgcctactgcaccacacaggtggagaggaacgcctgtctgttttgtaaagctcggaagctggatgataagttttaccagaagctgcggggccagttccccgatgccgtcttttggcaggagattagcgagatcttcagacagctgcagaagcaggccgccgagatctacaaccagagcctgatcgagctctactacgagatcttcatcaagggcaagggcattgccaacgcctcctccgtggagcactacctgagcgacgtgtgctacacaagagccgccgagctctttaagaacgccgctatcgcttccgggctgaggagcaagattaagagtaacttccggctcaaggagctgaagaacatgaagagcggcctgcccactacaaagagcgacaacttcccaattccactggtgaagcagaaggggggccagtacacagggttcgagatttccaaccacaacagcgactttattattaagatcccctttggcaggtggcaggtcaagaaggagattgacaagtacaggccctgggagaagtttgatttcgagcaggtgcagaagagccccaagcctatttccctgctgctgtccacacagcggcggaagaggaacaaggggtggtctaaggatgaggggaccgaggccgagattaagaaagtgatgaacggcgactaccagacaagctacatcgaggtcaagcggggcagtaagattggcgagaagagcgcctggatgctgaacctgagcattgacgtgccaaagattgataagggcgtggatcccagcatcatcggagggatcgatgtgggggtcaagagccccctcgtgtgcgccatcaacaacgccttcagcaggtacagcatctccgataacgacctgttccactttaacaagaagatgttcgcccggcggaggattttgctcaagaagaaccggcacaagcgggccggacacggggccaagaacaagctcaagcccatcactatcctgaccgagaagagcgagaggttcaggaagaagctcatcgagagatgggcctgcgagatcgccgatttctttattaagaacaaggtcggaacagtgcagatggagaacctcgagagcatgaagaggaaggaggattcctacttcaacattcggctgagggggttctggccctacgctgagatgcagaacaagattgagtttaagctgaagcagtacgggattgagatccggaaggtggcccccaacaacaccagcaagacctgcagcaagtgcgggcacctcaacaactacttcaacttcgagtaccggaagaagaacaagttcccacacttcaagtgcgagaagtgcaactttaaggagaacgccgattacaacgccgccctgaacatcagcaaccctaagctgaagagcactaaggaggagccc

SEQ ID NO: 482 - DNA, 1665 bp, Artificial Sequence
  Cas12f1 + random 26aa Encoding DNA
atggctggcggaccaggcgcaggtagtgctgcgccagtttcttcaacttcctccctgcccctggctgcgcttaacatgatggccaagaacacaattacaaagacactgaagctgaggatcgtgagaccatacaacagcgctgaggtcgagaagattgtggctgatgaaaagaacaacagggaaaagatcgccctcgagaagaacaaggataaggtgaaggaggcctgctctaagcacctgaaagtggccgcctactgcaccacacaggtggagaggaacgcctgtctgttttgtaaagctcggaagctggatgataagttttaccagaagctgcggggccagttccccgatgccgtcttttggcaggagattagcgagatcttcagacagctgcagaagcaggccgccgagatctacaaccagagcctgatcgagctctactacgagatcttcatcaagggcaagggcattgccaacgcctcctccgtggagcactacctgagcgacgtgtgctacacaagagccgccgagctctttaagaacgccgctatcgcttccgggctgaggagcaagattaagagtaacttccggctcaaggagctgaagaacatgaagagcggcctgcccactacaaagagcgacaacttcccaattccactggtgaagcagaaggggggccagtacacagggttcgagatttccaaccacaacagcgactttattattaagatcccctttggcaggtggcaggtcaagaaggagattgacaagtacaggccctgggagaagtttgatttcgagcaggtgcagaagagccccaagcctatttccctgctgctgtccacacagcggcggaagaggaacaaggggtggtctaaggatgaggggaccgaggccgagattaagaaagtgatgaacggcgactaccagacaagctacatcgaggtcaagcggggcagtaagattggcgagaagagcgcctggatgctgaacctgagcattgacgtgccaaagattgataagggcgtggatcccagcatcatcggagggatcgatgtgggggtcaagagccccctcgtgtgcgccatcaacaacgccttcagcaggtacagcatctccgataacgacctgttccactttaacaagaagatgttcgcccggcggaggattttgctcaagaagaaccggcacaagcgggccggacacggggccaagaacaagctcaagcccatcactatcctgaccgagaagagcgagaggttcaggaagaagctcatcgagagatgggcctgcgagatcgccgatttctttattaagaacaaggtcggaacagtgcagatggagaacctcgagagcatgaagaggaaggaggattcctacttcaacattcggctgagggggttctggccctacgctgagatgcagaacaagattgagtttaagctgaagcagtacgggattgagatccggaaggtggcccccaacaacaccagcaagacctgcagcaagtgcgggcacctcaacaactacttcaacttcgagtaccggaagaagaacaagttcccacacttcaagtgcgagaagtgcaactttaaggagaacgccgattacaacgccgccctgaacatcagcaaccctaagctgaagagcactaaggaggagccc

SEQ ID NO: 483 - DNA, 26 bp, Artificial Sequence
  CEP290 qPCR F#1
tggaccagaccctttgtagttatctt

SEQ ID NO: 484 - DNA, 24 bp, Artificial Sequence
  CEP290 qPCR R#1
tgagccagcaaaagcttttgagct

SEQ ID NO: 485 - DNA, 26 bp, Artificial Sequence
  CEP290 64 qPCR F#01
cttacatcctccttactgccacaaga

SEQ ID NO: 486 - DNA, 26 bp, Artificial Sequence
  CEP290 64 qPCR R#01
actgtggtcagaaaactcagctagtt

SEQ ID NO: 487 - DNA, 26 bp, Artificial Sequence
  inner F
tgtggcagccattattcctgtctcta

SEQ ID NO: 488 - DNA, 26 bp, Artificial Sequence
  inner R
gcaacacagtgagactctgtttcaaa

SEQ ID NO: 489 - DNA, 30 bp, Artificial Sequence
  right arm F
ggaactatgattcaagatgagatttgggta

SEQ ID NO: 490 - DNA, 24 bp, Artificial Sequence
  right arm R
ttggacacttcaactttgagctcc

SEQ ID NO: 491 - DNA, 26 bp, Artificial Sequence
  left arm F
tcttctgtggctatcatgagagcgtc

SEQ ID NO: 492 - DNA, 26 bp, Artificial Sequence
  left arm R
tgggtacaggggtaagagaaagggat